European Patent Application EP 4 545 564 A1, published April 30, 2025. Title: ANTIGEN-BINDING MOLECULE SPECIFICALLY BINDING TO DLL3 AND CD3, AND PHARMACEUTICAL USE THEREOF. Applicant: JIANGSU HENGRUI PHARMACEUTICALS CO., LTD. Application WO. The sequence listing filed with the application follows.

SEQUENCE LISTING (260 sequences)

SEQ ID NO: 1 - protein, 618 aa, Homo sapiens
MVSPRMSGLLSQTVILALIFLPQTRPAGVFELQIHSFGPGPGPGAPRSPCSARLPCRLFFRVCLKPGLSEEAAESPCALGAALSARGPVYTEQPGAPAPDLPLPDGLLQVPFRDAWPGTFSFIIETWREELGDQIGGPAWSLLARVAGRRRLAAGGPWARDIQRAGAWELRFSYRARCEPPAVGTACTRLCRPRSAPSRCGPGLRPCAPLEDECEAPLVCRAGCSPEHGFCEQPGECRCLEGWTGPLCTVPVSTSSCLSPRGPSSATTGCLVPGPGPCDGNPCANGGSCSETPRSFECTCPRGFYGLRCEVSGVTCADGPCFNGGLCVGGADPDSAYICHCPPGFQGSNCEKRVDRCSLQPCRNGGLCLDLGHALRCRCRAGFAGPRCEHDLDDCAGRACANGGTCVEGGGAHRCSCALGFGGRDCRERADPCAARPCAHGGRCYAHFSGLVCACAPGYMGARCEFPVHPDGASALPAAPPGLRPGDPQRYLLPPALGLLVAAGVAGAALLLVHVRRRGHSQDAGSRLLAGTPEPSVHALPDALNNLRTQEGSGDGPSSSVDWNRPEDVDPQGIYVISAPSIYAREVATPLFPPLHTGRAGQRQHLLFPYPSSILSVK

SEQ ID NO: 2 - protein, 618 aa, Macaca fascicularis
MVSPRMSRLLSQTVILALIFIPQARPAGVFELQIHSFGPGPGPGAPRSPCSARGPCRLFFRVCLKPGLSEEAAESPCALGAALSARGPVYTEQPEAPAPDLPLPNGLLQVPFRDAWPGTFSLIIETWREELGDQIGGPAWSLLARVTRRRRLAAGGPWARDIQRAGAWELRFSYRARCELPAVGTACTRLCRPRSAPSRCGPGLRPCAPLEDECEAPPVCRAGCSLEHGFCEQPGECRCLEGWTGPLCMVPVSTSSCLGLRGPSSTTTGCLVPGPGPCDGNPCANGGSCSETPGSFECTCPRGFYGLRCEVSGVTCADGPCFNGGLCVGGADPDSAYICHCPPGFQGSNCEKRVDRCSLQPCRNGGLCLDLGHALRCRCRAGFAGPRCEHDLDDCAGRACANGGTCVEGGGAHRCSCALGFGGRNCRERADPCAARPCAHGGRCYAHFSGLVCACAPGYMGARCEFPVHPDGVSALPAAPPGLRPGDPQRYLLPPALGLLVAAGVAGAALLLVHVRRRGHAQDAGSRLLAGTPEPSVHALPDALNNLRTQEGPGDVPSSSVDWNRPEDVDSRGIYVISAPSIYAREVAMPLFPPLHTGRAGQRQNLLFPFPSSILSVK

SEQ ID NO: 3 - protein, 589 aa, Rattus norvegicus
MVSLQVSSLPQTLILAFLLPQALPAGVFELQIHSFGPGPGPGTPRSPCNARGPCRLFFRVCLKPGVSQEAAESLCALGAALSTSGPVYTEQPGVPAAALSLPDGLVRVPFLDAWPGTFSLIIETWREQLGERAAGPAWNLLARVAGRRRLAAGAPWARDVQRTGAWELHFSYRARCEPPAVGAACARLCRSRSAPSRCGPGLRPCTPFPDECEAPRESLTVCRAGCSPEHGYCEEPDECHCLEGWTGPLCTVPVSTSSCLNSRVSGPAGTGCLLPGPGPCDGNPCANGGSCSETPGSFECACPRGFYGPRCEVSGVTCADGPCFNGGLCVGGEDPDSAYVCHCPPAFQGSNCERRVDRCSLQPCQNGGLCLDLGHALRCRCRAGFAGPRCEHDLDDCAGRACANGGTCVEGGGARRCSCALGFGGRDCRERADPCASRPCAHGGRCYAHFSGLVCACAPGYMGVRCEFAVRPDGADAVPAAPRGLRQADSQRFLLPPALGLLAAAALAGAALLLIHVRRRGPGRDTGTRLLSGTREPSVHTLPDALNNLRLQDGAGDGPTSSADWNHPEDGDSRSIYVIPAPSIYAREA

SEQ ID NO: 4 - protein, 592 aa, Mus musculus
MVSLQVSPLSQTLILAFLLPQALPAGVFELQIHSFGPGPGLGTPRSPCNARGPCRLFFRVCLKPGVSQEATESLCALGAALSTSVPVYTEHPGESAAALPLPDGLVRVPFRDAWPGTFSLVIETWREQLGEHAGGPAWNLLARVVGRRRLAAGGPWARDVQRTGTWELHFSYRARCEPPAVGAACARLCRSRSAPSRCGPGLRPCTPFPDECEAPSVCRPGCSPEHGYCEEPDECRCLEGWTGPLCTVPVSTSSCLNSRVPGPASTGCLLPGPGPCDGNPCANGGSCSETSGSFECACPRGFYGLRCEVSGVTCADGPCFNGGLCVGGEDPDSAYVCHCPPGFQGSNCEKRVDRCSLQPCQNGGLCLDLGHALRCRCRAGFAGPRCEHDLDDCAGRACANGGTCVEGGGSRRCSCALGFGGRDCRERADPCASRPCAHGGRCYAHFSGLVCACAPGYMGVRCEFAVRPDGADAVPAAPRGLRQADPQRFLLPPALGLLVAAGLAGAALLVIHVRRRGPGQDTGTRLLSGTREPSVHTLPDALNNLRLQDGAGDGPSSSADWNHPEDGDSRSIYVIPAPSIYAREDWLIQVLF

SEQ ID NO: 5 - protein, 723 aa, Homo sapiens
MGSRCALALAVLSALLCQVWSSGVFELKLQEFVNKKGLLGNRNCCRGGAGPPPCACRTFFRVCLKHYQASVSPEPPCTYGSAVTPVLGVDSFSLPDGGGADSAFSNPIRFPFGFTWPGTFSLIIEALHTDSPDDLATENPERLISRLATQRHLTVGEEWSQDLHSSGRTDLKYSYRFVCDEHYYGEGCSVFCRPRDDAFGHFTCGERGEKVCNPGWKGPYCTEPICLPGCDEQHGFCDKPGECKCRVGWQGRYCDECIRYPGCLHGTCQQPWQCNCQEGWGGLFCNQDLNYCTHHKPCKNGATCTNTGQGSYTCSCRPGYTGATCELGIDECDPSPCKNGGSCTDLENSYSCTCPPGFYGKICELSAMTCADGPCFNGGRCSDSPDGGYSCRCPVGYSGFNCEKKIDYCSSSPCSNGAKCVDLGDAYLCRCQAGFSGRHCDDNVDDCASSPCANGGTCRDGVNDFSCTCPPGYTGRNCSAPVSRCEHAPCHNGATCHERGHRYVCECARGYGGPNCQFLLPELPPGPAVVDLTEKLEGQGGPFPWVAVCAGVILVLMLLLGCAAVVVCVRLRLQKHRPPADPCRGETETMNNLANCQREKDISVSIIGATQIKNTNKKADFHGDHSADKNGFKARYPAVDYNLVQDLKGDDTAVRDAHSKRDTKCQPQGSSGEEKGTPTTLRGGEASERKRPDSGCSTSKDTKYQSVYVISEEKDECVIATEV

SEQ ID NO: 6 - protein, 685 aa, Homo sapiens
MAAASRSASGWALLLLVALWQQRAAGSGVFQLQLQEFINERGVLASGRPCEPGCRTFFRVCLKHFQAVVSPGPCTFGTVSTPVLGTNSFAVRDDSSGGGRNPLQLPFNFTWPGTFSLIIEAWHAPGDDLRPEALPPDALISKIAIQGSLAVGQNWLLDEQTSTLTRLRYSYRVICSDNYYGDNCSRLCKKRNDHFGHYVCQPDGNLSCLPGWTGEYCQQPICLSGCHEQNGYCSKPAECLCRPGWQGRLCNECIPHNGCRHGTCSTPWQCTCDEGWGGLFCDQDLNYCTHHSPCKNGATCSNSGQRSYTCTCRPGYTGVDCELELSECDSNPCRNGGSCKDQEDGYHCLCPPGYYGLHCEHSTLSCADSPCFNGGSCRERNQGANYACECPPNFTGSNCEKKVDRCTSNPCANGGQCLNRGPSRMCRCRPGFTGTYCELHVSDCARNPCAHGGTCHDLENGLMCTCPAGFSGRRCEVRTSIDACASSPCFNRATCYTDLSTDTFVCNCPYGFVGSRCEFPVGLPPSFPWVAVSLGVGLAVLLVLLGMVAVAVRQLRLRRPDDGSREAMNNLSDFQKDNLIPAAQLKNTNQKKELEVDCGLDKSNCGKQQNHTLDYNLAPGPLGRGTMPGKFPHSDKSLGEKAPLRLHSEKPECRISAICSPRDSMYQSVCLISEERNECVIATEV

SEQ ID NO: 7 - protein, 507 aa, synthetic construct
  REGION 1..507: note = His-hDLL3(ECD)
METDTLLLWVLLLWVPGSTGHHHHHHHHHHGGGGGSGGGGSAGVFELQIHSFGPGPGPGAPRSPCSARLPCRLFFRVCLKPGLSEEAAESPCALGAALSARGPVYTEQPGAPAPDLPLPDGLLQVPFRDAWPGTFSFIIETWREELGDQIGGPAWSLLARVAGRRRLAAGGPWARDIQRAGAWELRFSYRARCEPPAVGTACTRLCRPRSAPSRCGPGLRPCAPLEDECEAPLVCRAGCSPEHGFCEQPGECRCLEGWTGPLCTVPVSTSSCLSPRGPSSATTGCLVPGPGPCDGNPCANGGSCSETPRSFECTCPRGFYGLRCEVSGVTCADGPCFNGGLCVGGADPDSAYICHCPPGFQGSNCEKRVDRCSLQPCRNGGLCLDLGHALRCRCRAGFAGPRCEHDLDDCAGRACANGGTCVEGGGAHRCSCALGFGGRDCRERADPCAARPCAHGGRCYAHFSGLVCACAPGYMGARCEFPVHPDGASALPAAPPGLRPGDPQRYL

SEQ ID NO: 8 - protein, 727 aa, synthetic construct
  REGION 1..727: note = Fc-hDLL3(ECD)
METDTLLLWVLLLWVPGSTGEPKSSDKTHTCPPCPAPELLGGPSVFLFPPKPKDTLMISRTPEVTCVVVDVSHEDPEVKFNWYVDGVEVHNAKTKPREEQYNSTYRVVSVLTVLHQDWLNGKEYKCKVSNKALPAPIEKTISKAKGQPREPQVYTLPPSRDELTKNQVSLTCLVKGFYPSDIAVEWESNGQPENNYKTTPPVLDSDGSFFLYSKLTVDKSRWQQGNVFSCSVMHEALHNHYTQKSLSLSPGGGGGSGGGGSAGVFELQIHSFGPGPGPGAPRSPCSARLPCRLFFRVCLKPGLSEEAAESPCALGAALSARGPVYTEQPGAPAPDLPLPDGLLQVPFRDAWPGTFSFIIETWREELGDQIGGPAWSLLARVAGRRRLAAGGPWARDIQRAGAWELRFSYRARCEPPAVGTACTRLCRPRSAPSRCGPGLRPCAPLEDECEAPLVCRAGCSPEHGFCEQPGECRCLEGWTGPLCTVPVSTSSCLSPRGPSSATTGCLVPGPGPCDGNPCANGGSCSETPRSFECTCPRGFYGLRCEVSGVTCADGPCFNGGLCVGGADPDSAYICHCPPGFQGSNCEKRVDRCSLQPCRNGGLCLDLGHALRCRCRAGFAGPRCEHDLDDCAGRACANGGTCVEGGGAHRCSCALGFGGRDCRERADPCAARPCAHGGRCYAHFSGLVCACAPGYMGARCEFPVHPDGASALPAAPPGLRPGDPQRYL

SEQ ID NO: 9 - protein, 514 aa, synthetic construct
  REGION 1..514: note = hDLL3(ECD)-strep twin
METDTLLLWVLLLWVPGSTGAGVFELQIHSFGPGPGPGAPRSPCSARLPCRLFFRVCLKPGLSEEAAESPCALGAALSARGPVYTEQPGAPAPDLPLPDGLLQVPFRDAWPGTFSFIIETWREELGDQIGGPAWSLLARVAGRRRLAAGGPWARDIQRAGAWELRFSYRARCEPPAVGTACTRLCRPRSAPSRCGPGLRPCAPLEDECEAPLVCRAGCSPEHGFCEQPGECRCLEGWTGPLCTVPVSTSSCLSPRGPSSATTGCLVPGPGPCDGNPCANGGSCSETPRSFECTCPRGFYGLRCEVSGVTCADGPCFNGGLCVGGADPDSAYICHCPPGFQGSNCEKRVDRCSLQPCRNGGLCLDLGHALRCRCRAGFAGPRCEHDLDDCAGRACANGGTCVEGGGAHRCSCALGFGGRDCRERADPCAARPCAHGGRCYAHFSGLVCACAPGYMGARCEFPVHPDGASALPAAPPGLRPGDPQRYLWSHPQFEKGGGSGGGSGGSAWSHPQFEK

SEQ ID NO: 10 - protein, 514 aa, synthetic construct
  REGION 1..514: note = cynoDLL3(ECD)-strep twin
METDTLLLWVLLLWVPGSTGAGVFELQIHSFGPGPGPGAPRSPCSARGPCRLFFRVCLKPGLSEEAAESPCALGAALSARGPVYTEQPEAPAPDLPLPNGLLQVPFRDAWPGTFSLIIETWREELGDQIGGPAWSLLARVTRRRRLAAGGPWARDIQRAGAWELRFSYRARCELPAVGTACTRLCRPRSAPSRCGPGLRPCAPLEDECEAPPVCRAGCSLEHGFCEQPGECRCLEGWTGPLCMVPVSTSSCLGLRGPSSTTTGCLVPGPGPCDGNPCANGGSCSETPGSFECTCPRGFYGLRCEVSGVTCADGPCFNGGLCVGGADPDSAYICHCPPGFQGSNCEKRVDRCSLQPCRNGGLCLDLGHALRCRCRAGFAGPRCEHDLDDCAGRACANGGTCVEGGGAHRCSCALGFGGRNCRERADPCAARPCAHGGRCYAHFSGLVCACAPGYMGARCEFPVHPDGVSALPAAPPGLRPGDPQRYLWSHPQFEKGGGSGGGSGGSAWSHPQFEK

SEQ ID NO: 11 - protein, 514 aa, synthetic construct
  REGION 1..514: note = mouDLL3(ECD)-strep twin
METDTLLLWVLLLWVPGSTGAGVFELQIHSFGPGPGLGTPRSPCNARGPCRLFFRVCLKPGVSQEATESLCALGAALSTSVPVYTEHPGESAAALPLPDGLVRVPFRDAWPGTFSLVIETWREQLGEHAGGPAWNLLARVVGRRRLAAGGPWARDVQRTGTWELHFSYRARCEPPAVGAACARLCRSRSAPSRCGPGLRPCTPFPDECEAPSVCRPGCSPEHGYCEEPDECRCLEGWTGPLCTVPVSTSSCLNSRVPGPASTGCLLPGPGPCDGNPCANGGSCSETSGSFECACPRGFYGLRCEVSGVTCADGPCFNGGLCVGGEDPDSAYVCHCPPGFQGSNCEKRVDRCSLQPCQNGGLCLDLGHALRCRCRAGFAGPRCEHDLDDCAGRACANGGTCVEGGGSRRCSCALGFGGRDCRERADPCASRPCAHGGRCYAHFSGLVCACAPGYMGVRCEFAVRPDGADAVPAAPRGLRQADPQRFLWSHPQFEKGGGSGGGSGGSAWSHPQFEK

SEQ ID NO: 12 - protein, 120 aa, synthetic construct
  REGION 1..120: note = mAb6
EVQLQQSGPVLVKPGASVKMSCKASGYTFTDYYMNWVKQSHGKSLEWIGIINPYSGVTIYNHKFKGKATLTVDKSSNTAYMELNSLTSEDSAVYYCARQDSLLDYAMDYWGQGTSVTVSS

SEQ ID NO: 13 - protein, 107 aa, synthetic construct
  REGION 1..107: note = mAb6
DILMTQSPSSMSVSLGDTVSITCHASQGISGNMGWLQQKPGKSFKGLIYHGANLEDGVPSRFSGSGSGADYSLTISSLESEDFADYYCVQYAQFPYTFGGGTKLEIK

SEQ ID NO: 14 - protein, 121 aa, synthetic construct
  REGION 1..121: note = mAb98
EVQLVESGGGLVKPGGSLKLSCAASGFTFSDYGIHWVRQAPEKGLEWVAYISSGGYTIYYADTVKGRFTISRDNAKNTLFLQMTSLRSEDTAMYYCARGDYDDIFYTMDYWGQGTSVTVSS

SEQ ID NO: 15 - protein, 107 aa, synthetic construct
  REGION 1..107: note = mAb98
DIQMTQTTSSLSASLGDRVTISCRASRDITKFLNWYQQKPDGTVKLLIYYTSRLHSGVPSRFSGSGSGTDYSLTISNLDQEDIATYFCQQGNTLPWTFGGGTKLDIK

SEQ ID NO: 16 - protein, 124 aa, synthetic construct
  REGION 1..124: note = mAb110
EVQLQQSGPVLVKPGASVKMSCKTSGYTFTDYYMNWVKQSHGKSLEWIGIINPYNGGTSYTQKFKGKATLTVDKSSSTAYMELNSLTSEDSTVYFCARHFYDSSYLTYSTMDYWGQGTSVTVSS

SEQ ID NO: 17 - protein, 107 aa, synthetic construct
  REGION 1..107: note = mAb110
NIVMTQSPKSMSMSVGERVTLSCKASENVGIFVSWYQQKPKQSPKLLIYGASNRYTGVPDRFTGSGSATDFTLTISSVQAEDLADYYCGQSHSYPLTFGTGTKLELK

SEQ ID NO: 18 - protein, 122 aa, synthetic construct
  REGION 1..122: note = mAb30
EVRLQQFGPVLVKPGASVKMSCKASGYTFTDYYMNWVKQSHGKSLEWIGIINPYNGDTSYNQKFRGKATLTVDKSSSTAYMELNSLTSEDSAVYYCARYHYGPHLEGYFDVWGTGTTLTVSS

SEQ ID NO: 19 - protein, 106 aa, synthetic construct
  REGION 1..106: note = mAb30
DIVMTQSPKSMSMSVGERVTLSCKASENVGYVSWYQQKPEQSPKLLIYGASNRYTGVPDRFTGSGSATDFTLTISSVQAEDLADYHCGQSYSYPLTFGSGTKLEIK

SEQ ID NO: 20 - protein, 5 aa, Mus musculus
  REGION 1..5: note = mAb6 mAb110 mAb30 HCDR1
DYYMN

SEQ ID NO: 21 - protein, 17 aa, Mus musculus
  REGION 1..17: note = mAb6 HCDR2
IINPYSGVTIYNHKFKG

SEQ ID NO: 22 - protein, 11 aa, Mus musculus
  REGION 1..11: note = mAb6 HCDR3
QDSLLDYAMDY

SEQ ID NO: 23 - protein, 11 aa, Mus musculus
  REGION 1..11: note = mAb6 LCDR1
HASQGISGNMG

SEQ ID NO: 24 - protein, 7 aa, Mus musculus
  REGION 1..7: note = mAb6 LCDR2
HGANLED

SEQ ID NO: 25 - protein, 9 aa, Mus musculus
  REGION 1..9: note = mAb6 LCDR3
VQYAQFPYT

SEQ ID NO: 26 - protein, 5 aa, Mus musculus
  REGION 1..5: note = mAb98 HCDR1
DYGIH

SEQ ID NO: 27 - protein, 17 aa, Mus musculus
  REGION 1..17: note = mAb98 HCDR2
YISSGGYTIYYADTVKG

SEQ ID NO: 28 - protein, 12 aa, Mus musculus
  REGION 1..12: note = mAb98 HCDR3
GDYDDIFYTMDY

SEQ ID NO: 29 - protein, 11 aa, Mus musculus
  REGION 1..11: note = mAb98 LCDR1
RASRDITKFLN

SEQ ID NO: 30 - protein, 7 aa, Mus musculus
  REGION 1..7: note = mAb98 LCDR2
YTSRLHS

SEQ ID NO: 31 - protein, 9 aa, Mus musculus
  REGION 1..9: note = mAb98 LCDR3
QQGNTLPWT

SEQ ID NO: 32 - protein, 17 aa, Mus musculus
  REGION 1..17: note = mAb110 HCDR2
IINPYNGGTSYTQKFKG

SEQ ID NO: 33 - protein, 15 aa, Mus musculus
  REGION 1..15: note = mAb110 HCDR3
HFYDSSYLTYSTMDY

SEQ ID NO: 34 - protein, 11 aa, Mus musculus
  REGION 1..11: note = mAb110 LCDR1
KASENVGIFVS

SEQ ID NO: 35 - protein, 7 aa, Mus musculus
  REGION 1..7: note = mAb110 mAb30 LCDR2
GASNRYT

SEQ ID NO: 36 - protein, 9 aa, Mus musculus
  REGION 1..9: note = mAb110 LCDR3
GQSHSYPLT

SEQ ID NO: 37 - protein, 17 aa, Mus musculus
  REGION 1..17: note = mAb30 HCDR2
IINPYNGDTSYNQKFRG

SEQ ID NO: 38 - protein, 13 aa, Mus musculus
  REGION 1..13: note = mAb30 HCDR3
YHYGPHLEGYFDV

SEQ ID NO: 39 - protein, 10 aa, Mus musculus
  REGION 1..10: note = mAb30 LCDR1
KASENVGYVS

SEQ ID NO: 40 - protein, 9 aa, Mus musculus
  REGION 1..9: note = mAb30 LCDR3
GQSYSYPLT

SEQ ID NO: 41 - protein, 330 aa, Homo sapiens [sequence omitted]

SEQ ID NO: 42 - protein, 107 aa, Homo sapiens [sequence omitted]

SEQ ID NO: 43 - protein, 120 aa, synthetic construct
  REGION 1..120: note = hu6 VH1
EVQLVQSGAEVKKPGASVKVSCKASGYTFTDYYMNWVRQAPGQRLEWMGIINPYSGVTIYNHKFKGRVTITVDKSASTAYMELSSLRSEDTAVYYCARQDSLLDYAMDYWGQGTTVTVSS

SEQ ID NO: 44 - protein, 120 aa, synthetic construct
  REGION 1..120: note = hu6 VH2
EVQLVQSGAEVKKPGASVKVSCKASGYTFTDYYMNWVRQAPGQRLEWMGIINPYSGVTIYNHKFKGRVTLTVDKSANTAYMELSSLRSEDTAVYYCARQDSLLDYAMDYWGQGTTVTVSS

SEQ ID NO: 45 - protein, 120 aa, synthetic construct
  REGION 1..120: note = hu6 VH3
EVQLVQSGAEVKKPGASVKVSCKASGYTFTDYYMNWVRQAPGQRLEWIGIINPYSGVTIYNHKFKGRATLTVDKSANTAYMELSSLRSEDTAVYYCARQDSLLDYAMDYWGQGTTVTVSS

SEQ ID NO: 46 - protein, 120 aa, synthetic construct
  REGION 1..120: note = hu6 VH4
EVQLVQSGAEVKKPGASVKVSCKASGYTFTDYYMNWVRQAPGKRLEWMGIINPYSGVTIYNHKFKGRVTLTVDKSANTAYMELSSLRSEDTAVYYCARQDSLLDYAMDYWGQGTTVTVSS

SEQ ID NO: 47 - protein, 120 aa, synthetic construct
  REGION 1..120: note = hu6 VH5
EVQLVQSGSELKKPGASVKVSCKASGYTFTDYYMNWVRQAPGQGLEWMGIINPYSGVTIYNHKFKGRFVLSVDKSVSTAYLQISSLKAEDTAVYYCARQDSLLDYAMDYWGQGTTVTVSS

SEQ ID NO: 48 - protein, 120 aa, synthetic construct
  REGION 1..120: note = hu6 VH6
EVQLVQSGSELKKPGASVKVSCKASGYTFTDYYMNWVRQAPGQGLEWMGIINPYSGVTIYNHKFKGRFVLSVDKSSNTAYLQISSLKAEDTAVYYCARQDSLLDYAMDYWGQGTTVTVSS

SEQ ID NO: 49 - protein, 120 aa, synthetic construct
  REGION 1..120: note = hu6 VH7
EVQLVESGGGLVQPGGSLKLSCAASGYTFTDYYMNWVRQASGKGLEWVGIINPYSGVTIYNHKFKGRFTLSVDKSKNTAYLQMNSLKTEDTAVYYCARQDSLLDYAMDYWGQGTTVTVSS

SEQ ID NO: 50 - protein, 120 aa, synthetic construct
  REGION 1..120: note = hu6VH8
QVQLVQSGAEVKKPGASVKVSCKASGYTFTDYYMNWVRQAPGQRLEWMGIINPYSGVTIYNHKFKGRVTITRDTSASTAYMELSSLRSEDTAVYYCARQDSLLDYAMDYWGQGTTVTVSS

SEQ ID NO: 51 - protein, 120 aa, synthetic construct
  REGION 1..120: note = hu6VH9
QVQLVQSGSELKKPGASVKVSCKASGYTFTDYYMNWVRQAPGQGLEWMGIINPYSGVTIYNHKFKGRFVFSLDTSVSTAYLQISSLKAEDTAVYYCARQDSLLDYAMDYWGQGTTVTVSS

SEQ ID NO: 52 - protein, 120 aa, synthetic construct
  REGION 1..120: note = hu6VH10
EVQLVESGGGLVQPGGSLKLSCAASGFTFSDYYMNWVRQASGKGLEWVGIINPYSGVTIYNHKFKGRFTISRDDSKNTAYLQMNSLKTEDTAVYYCTRQDSLLDYAMDYWGQGTTVTVSS

SEQ ID NO: 53 - protein, 120 aa, synthetic construct
  REGION 1..120: note = hu6VH11
EVQLVQSGSELKKPGASVKVSCKASGYTFTDYYMNWVKQAPGQGLEWMGIINPYSGVTIYNHKFKGRFVLSVDKSSNTAYLQISSLKAEDTAVYYCARQDSLLDYAMDYWGQGTTVTVSS

SEQ ID NO: 54 - protein, 120 aa, synthetic construct
  REGION 1..120: note = hu6VH12
EVQLVQSGSELKKPGASVKVSCKASGYTFTDYYMNWVRQAPGQGLEWMGIINPYSGVTIYNHKFKGRFALSVDKSSNTAYLQISSLKAEDTAVYYCARQDSLLDYAMDYWGQGTTVTVSS

SEQ ID NO: 55 - protein, 120 aa, synthetic construct
  REGION 1..120: note = hu6VH13
EVQLVQSGSELKKPGASVKVSCKASGYTFTDYYMNWVKQAPGQGLEWMGIINPYSGVTIYNHKFKGRFALSVDKSSNTAYLQISSLKAEDTAVYYCARQDSLLDYAMDYWGQGTTVTVSS

SEQ ID NO: 56 - protein, 120 aa, synthetic construct
  REGION 1..120: note = hu6VH14
EVQLVQSGSELKKPGASVKVSCKASGYTFTDYYMNWVRQAPGQGLEWMGIINPYSGVTTYNHKFKGRFALSVDKSSNTAYLQISSLKAEDTAVYYCARQDSLLDYAMDYWGQGTTVTVSS

SEQ ID NO: 57 - protein, 120 aa, synthetic construct
  REGION 1..120: note = hu6VH15
EVQLQQSGSELKKPGASVKVSCKASGYTFTDYYMNWVRQAPGQGLEWMGIINPYSGSTIYNHKFKGRFALSVDKSSNTAYLQISSLKAEDTAVYYCARQDSLLDYAMDYWGQGTTVTVSS

SEQ ID NO: 58 - protein, 107 aa, synthetic construct
  REGION 1..107: note = hu6 VL1
DIQMTQSPSSLSASVGDRVTITCHASQGISGNMGWLQQKPGKAPKGLIYHGANLEDGVPSRFSGSGSGTDFTLTISSLQPEDFATYYCVQYAQFPYTFGGGTKVEIK

SEQ ID NO: 59 - protein, 107 aa, synthetic construct
  REGION 1..107: note = hu6 VL2
DIQMTQSPSSLSASVGDRVTITCHASQGISGNMGWLQQKPGKAPKGLIYHGANLEDGVPSRFSGSGSGADYTLTISSLQPEDFATYYCVQYAQFPYTFGGGTKVEIK

SEQ ID NO: 60 - protein, 107 aa, synthetic construct
  REGION 1..107: note = hu6 VL3
DIQMTQSPSSLSASVGDRVTITCHASQGISGNMGWLQQKPGKSFKGLIYHGANLEDGVPSRFSGSGSGADYTLTISSLQPEDFATYYCVQYAQFPYTFGGGTKVEIK

SEQ ID NO: 61 - protein, 107 aa, synthetic construct
  REGION 1..107: note = hu6 VL4
DIQMTQSPSSLSASVGDRVTITCHASQGISGNMGWLQQKPGKAPKGLIYHGANLEDGVPSRFSGSGSGADYTLTISSLQPEDFADYYCVQYAQFPYTFGGGTKVEIK

SEQ ID NO: 62 - protein, 107 aa, synthetic construct
  REGION 1..107: note = hu6VL5
DIQMTQSPSSLSASVGDRVTITCHASQGISGNMGWFQQKPGKAPKSLIYHGANLEDGVPSRFSGSGSGTDFTLTISSLQPEDFATYYCVQYAQFPYTFGGGTKVEIK

SEQ ID NO: 63 - protein, 107 aa, synthetic construct
  REGION 1..107: note = hu6VL6
DIQMTQSPSSLSASVGDRVTITCHASQGISGNMGWLQQKPGKAPKGLIYHGANLEEGVPSRFSGSGSGADYTLTISSLQPEDFADYYCVQYAQFPYTFGGGTKVEIK

SEQ ID NO: 64 - protein, 107 aa, synthetic construct
  REGION 1..107: note = hu6VL7
DIQMTQSPSSLSASVGDRVTITCHASQGISGNMGWLQQKPGKAPKGLIYHGANLESGVPSRFSGSGSGADYTLTISSLQPEDFADYYCVQYAQFPYTFGGGTKVEIK

SEQ ID NO: 65 - protein, 107 aa, synthetic construct
  REGION 1..107: note = hu6VL8
DIQMTQSPSSLSASVGDRVTITCHASQGISGNMGWLQQKPGKAPKGLIYHGANLEEGVPSRFSGSGSGADYTLTISSLQPEDFADYYCVQYAQYPYTFGGGTKVEIK

SEQ ID NO: 66 - protein, 107 aa, synthetic construct
  REGION 1..107: note = hu6VL9
NIQMTQSPSSLSASVGDRVTITCHASQGISGNMGWLQQKPGKAPKGLIYHGRNLEEGVPSRFSGSGSGADYTLTISSLQPEDFADYYCVQYAQYPYTFGGGTKVEIK

SEQ ID NO: 67 - protein, 107 aa, synthetic construct
  REGION 1..107: note = hu6VL10
EIVLTQSPATLSLSPGERATLSCHASQGISGNMGWLQQKPGKAPRGLIYHGANLEEGIPARFSGSGSGADYTLTISRLQPEDFADYYCVQYAQFPYTFGGGTKVEIK

SEQ ID NO: 68 - protein, 107 aa, synthetic construct
  REGION 1..107: note = hu6VL11
EIVLTQSPATLSLSPGERATLSCHASQGISGNMGWYQQKPGQAPRLLIYHGANLEEGIPARFSGSGSGTDFTLTISRLEPEDFAVYYCVQYAQFPYTFGGGTKVEIK

SEQ ID NO: 69 - protein, 16 aa, synthetic construct
  REGION 1..16: note = hu6VH14 HCDR2
INPYSGVTTYNHKFKG

SEQ ID NO: 70 - protein, 16 aa, synthetic construct
  REGION 1..16: note = hu6VH15 HCDR2
INPYSGSTIYNHKFKG

SEQ ID NO: 71 - protein, 7 aa, synthetic construct
  REGION 1..7: note = hu6VL6/VL8/VL10 LCDR2
HGANLEE

SEQ ID NO: 72 - protein, 7 aa, synthetic construct
  REGION 1..7: note = hu6VL7 LCDR2
HGANLES

SEQ ID NO: 73 - protein, 7 aa, synthetic construct
  REGION 1..7: note = hu6VL9 LCDR2
HGRNLEE

SEQ ID NO: 74 - protein, 9 aa, synthetic construct
  REGION 1..9: note = hu6VL8/VL9 LCDR3
VQYAQYPYT

SEQ ID NO: 75 - protein, 107 aa, synthetic construct
  REGION 1..107: note = hu98VL1
DIQMTQSPSSLSASVGDRVTITCRASRDITKFLNWYQQKPGKAPKLLIYYTSRLHSGVPSRFSGSGSGTDFTLTISSLQPEDFATYYCQQGNTLPWTFGGGTKVEIK

SEQ ID NO: 76 - protein, 107 aa, synthetic construct
  REGION 1..104: note = hu98VL2
DIQMTQSPSSLSASVGDRVTITCRASRDITKFLNWYQQKPGKAVKLLIYYTSRLHSGVPSRFSGSGSGTDYTLTISSLQPEDFATYYCQQGNTLPWTFGGGTKVEIK

SEQ ID NO: 77 - protein, 107 aa, synthetic construct
  REGION 1..107: note = hu98VL3
DIQMTQSPSSLSASVGDRVTITCRASRDITKFLNWYQQKPGGAVKLLIYYTSRLHSGVPSRFSGSGSGTDYTLTISSLQPEDFATYYCQQGNTLPWTFGGGTKVEIK

SEQ ID NO: 78 - protein, 121 aa, synthetic construct
  REGION 1..121: note = hu98VH1
EVQLVESGGGLVQPGGSLRLSCAASGFTFSDYGIHWVRQAPGKGLEWVAYISSGGYTIYYADTVKGRFTISRDNAKNSLYLQMNSLRAEDTAVYYCARGDYDDIFYTMDYWGQGTTVTVSS

SEQ ID NO: 79 - protein, 121 aa, synthetic construct
  REGION 1..121: note = hu98VH2
EVQLVESGGGLVQPGGSLRLSCAASGFTFSDYGIHWVRQAPGKGLEWVAYISSGGYTIYYADTVKGRFTISRDNAKNSLYLQMNSLRAEDTAVYYCARGDYEDIFYTMDYWGQGTTVTVSS

SEQ ID NO: 80 - protein, 121 aa, synthetic construct
  REGION 1..121: note = hu98VH3
EVQLVESGGGLVQPGGSLRLSCAASGFTFSDYGMHWVRQAPGKGLEWVAYISSGGYTIYYADTVKGRFTISRDNAKNSLYLQMNSLRAEDTAVYYCARGDYEDIFYTMDYWGQGTTVTVSS

SEQ ID NO: 81 - protein, 121 aa, synthetic construct
  REGION 1..121: note = hu98VH4
EVQLVESGGGLVQPGGSLRLSCAASGFTFSDYGIHWVRQAPGKGLEWVAYISSGGYTSYYADTVKGRFTISRDNAKNSLYLQMNSLRAEDTAVYYCARGDYEDIFYTMDYWGQGTTVTVSS

SEQ ID NO: 82 - protein, 121 aa, synthetic construct
  REGION 1..121: note = hu98VH5
EVQLVESGGGLVQPGGSLRLSCAASGFTFSDYGMHWVRQAPGKGLEWVAYISSGGYTSYYADTVKGRFTISRDNAKNSLYLQMNSLRAEDTAVYYCARGDYEDIFYTMDYWGQGTTVTVSS

SEQ ID NO: 83 - protein, 12 aa, synthetic construct
  REGION 1..12: note = hu98VH2/VH3/VH4/VH5 HCDR3
GDYEDIFYTMDY

SEQ ID NO: 84 - protein, 5 aa, synthetic construct
  REGION 1..5: note = hu98VH3/VH5 HCDR1
DYGMH

SEQ ID NO: 85 - protein, 17 aa, synthetic construct
  REGION 1..17: note = hu98VH4/VH5 HCDR2
YISSGGYTSYYADTVKG

SEQ ID NO: 86 - protein, 107 aa, synthetic construct
  REGION 1..107: note = hu110VL1
DIVMTQSPDSLAVSLGERATINCKASENVGIFVSWYQQKPGQSPKLLIYGASNRYTGVPDRFSGSGSATDFTLTISSLQAEDVAVYYCGQSHSYPLTFGQGTKLEIK

SEQ ID NO: 87 - protein, 107 aa, synthetic construct
  REGION 1..107: note = hu110VL2
NIVMTQSPKSLAVSLGERATINCKASENVGIFVSWYQQKPGQSPKLLIYGASNRYTGVPDRFSGSGSATDFTLTISSLQAEDVADYYCGQSHSYPLTFGQGTKLEIK

SEQ ID NO: 88 - protein, 107 aa, synthetic construct
  REGION 1..107: note = hu110VL3
DIVMTQSPDSLAVSLGERATINCKASENVGIFVSWYQQKPGQPPKLLIYGASNRYTGVPDRFSGSGSGTDFTLTISSLQAEDVAVYYCGQSHSYPLTFGQGTKLEIK

SEQ ID NO: 89 - protein, 124 aa, synthetic construct
  REGION 1..124: note = hu110VH1
EVQLVQSGAEVKKPGASVKVSCKASGYTFTDYYMNWVRQAPGQRLEWMGIINPYNGGTSYTQKFKGRVTITVDKSASTAYMELSSLRSEDTAVYYCARHFYDSSYLTYSTMDYWGQGTTVTVSS

SEQ ID NO: 90 - protein, 124 aa, synthetic construct
  REGION 1..124: note = hu110VH2
EVQLVQSGAEVKKPGASVKVSCKTSGYTFTDYYMNWVRQAPGQSLEWMGIINPYNGGTSYTQKFKGRVTITVDKSASTAYMELSSLRSEDTAVYYCARHFYDSSYLTYSTMDYWGQGTTVTVSS

SEQ ID NO: 91 - protein, 124 aa, synthetic construct
  REGION 1..124: note = hu110VH3
EVQLVQSGAEVKKPGASVKVSCKTSGYTFTDYYMNWVRQAPGQSLEWMGIINPYQGGTSYTQKFKGRVTITVDKSASTAYMELSSLRSEDTAVYYCARHFYDSSYLTYSTMDYWGQGTTVTVSS

SEQ ID NO: 92 - protein, 124 aa, synthetic construct
  REGION 1..124: note = hu110VH4
EVQLVQSGAEVKKPGASVKVSCKTSGYTFTDYYMNWVRQAPGQSLEWMGIINPYSGGTSYTQKFKGRVTITVDKSASTAYMELSSLRSEDTAVYYCARHFYDSSYLTYSTMDYWGQGTTVTVSS

SEQ ID NO: 93 - protein, 124 aa, synthetic construct
  REGION 1..124: note = hu110VH5
EVQLVQSGAEVKKPGASVKVSCKTSGYTFTDYYMNWVRQAPGQSLEWMGIINPYTGGTSYTQKFKGRVTITVDKSASTAYMELSSLRSEDTAVYYCARHFYDSSYLTYSTMDYWGQGTTVTVSS

SEQ ID NO: 94 - protein, 124 aa, synthetic construct
  REGION 1..124: note = hu110VH6
EVQLVQSGAEVKKPGASVKVSCKTSGYTFTDYYMNWVRQAPGQSLEWMGIINPYNVGTSYTQKFKGRVTITVDKSASTAYMELSSLRSEDTAVYYCARHFYDSSYLTYSTMDYWGQGTTVTVSS

SEQ ID NO: 95 - protein, 124 aa, synthetic construct
  REGION 1..124: note = hu110VH7
QVQLVQSGAEVKKPGASVKVSCKASGYTFTDYYMNWVRQAPGQRLEWMGIINPYNGGTSYTQKFKGRVTITRDTSASTAYMELSSLRSEDTAVYYCARHFYDSSYLTYSTMDYWGQGTTVTVSS

SEQ ID NO: 96 - protein, 17 aa, synthetic construct
  REGION 1..17: note = hu110VH3 HCDR2
IINPYQGGTSYTQKFKG

SEQ ID NO: 97 - protein, 17 aa, synthetic construct
  REGION 1..17: note = hu110VH4 HCDR2
IINPYSGGTSYTQKFKG

SEQ ID NO: 98 - protein, 17 aa, synthetic construct
  REGION 1..17: note = hu110VH5 HCDR2
IINPYTGGTSYTQKFKG

SEQ ID NO: 99 - protein, 17 aa, synthetic construct
  REGION 1..17: note = hu110VH6 HCDR2
IINPYNVGTSYTQKFKG

SEQ ID NO: 100 - protein, 106 aa, synthetic construct
  REGION 1..106: note = hu30VL1
DIVMTQSPDSLAVSLGERATINCKASENVGYVSWYQQKPGQPPKLLIYGASNRYTGVPDRFSGSGSGTDFTLTISSLQAEDVAVYYCGQSYSYPLTFGQGTKLEIK

SEQ ID NO: 101 - protein, 106 aa, synthetic construct
  REGION 1..106: note = hu30VL2
DIVMTQSPDSLAVSLGERATINCKASENVGYVSWYQQKPGQPPKLLIYGASNRYTGVPDRFSGSGSATDFTLTISSLQAEDVAVYHCGQSYSYPLTFGQGTKLEIK

SEQ ID NO: 102 - protein, 106 aa, synthetic construct
  REGION 1..106: note = hu30VL3
DIVMTQSPKSLAVSLGERATINCKASENVGYVSWYQQKPGQSPKLLIYGASNRYTGVPDRFSGSGSATDFTLTISSLQAEDVAVYHCGQSYSYPLTFGQGTKLEIK

SEQ ID NO: 103 - protein, 106 aa, synthetic construct
  REGION 1..106: note = hu30VL4
DIQMTQSPSSLSASVGDRVTITCKASENVGYVSWYQQKPGKAPKLLIYGASNRYTGVPSRFSGSGSGTDFTLTISSLQPEDFATYYCGQSYSYPLTFGQGTKLEIK

SEQ ID NO: 104 - protein, 106 aa, synthetic construct
  REGION 1..106: note = hu30VL5
DIQMTQSPSSLSASVGDRVTITCKASENVGYVSWYQQKPGKSPKLLIYGASNRYTGVPDRFSGSGSGTDFTLTISSLQPEDFATYYCGQSYSYPLTFGSGTKLEIK

SEQ ID NO: 105 - protein, 122 aa, synthetic construct
  REGION 1..122: note = hu30VH1
EVQLVQSGAEVKKPGASVKVSCKASGYTFTDYYMNWVRQAPGQSLEWMGIINPYNGDTSYNQKFRGRVTITVDKSASTAYMELSSLRSEDTAVYYCARYHYGPHLEGYFDVWGQGTTVTVSS

SEQ ID NO: 106 - protein, 122 aa, synthetic construct
  REGION 1..122: note = hu30VH2
EVRLVQSGAEVKKPGASVKVSCKASGYTFTDYYMNWVRQAPGQSLEWMGIINPYNGDTSYNQKFRGRVTLTVDKSASTAYMELSSLRSEDTAVYYCARYHYGPHLEGYFDVWGQGTTVTVSS

SEQ ID NO: 107 - protein, 122 aa, synthetic construct
  REGION 1..122: note = hu30VH3
EVRLVQSGAEVKKPGASVKVSCKASGYTFTDYYMNWVRQAPGQSLEWMGIINPYQGDTSYNQKFRGRVTLTVDKSASTAYMELSSLRSEDTAVYYCARYHYGPHLEGYFDVWGQGTTVTVSS

SEQ ID NO: 108 - protein, 122 aa, synthetic construct
  REGION 1..122: note = hu30VH4
EVRLVQSGAEVKKPGASVKVSCKASGYTFTDYYMNWVRQAPGQSLEWMGIINPYSGDTSYNQKFRGRVTLTVDKSASTAYMELSSLRSEDTAVYYCARYHYGPHLEGYFDVWGQGTTVTVSS

SEQ ID NO: 109 - protein, 122 aa, synthetic construct
  REGION 1..122: note = hu30VH5
EVRLVQSGAEVKKPGASVKVSCKASGYTFTDYYMNWVRQAPGQSLEWMGIINPYTGDTSYNQKFRGRVTLTVDKSASTAYMELSSLRSEDTAVYYCARYHYGPHLEGYFDVWGQGTTVTVSS

SEQ ID NO: 110 - protein, 122 aa, synthetic construct
  REGION 1..122: note = hu30VH6
EVRLVQSGAEVKKPGASVKVSCKASGYTFTDYYMNWVRQAPGQSLEWMGIINPYNVDTSYNQKFRGRVTLTVDKSASTAYMELSSLRSEDTAVYYCARYHYGPHLEGYFDVWGQGTTVTVSS

SEQ ID NO: 111 - protein, 122 aa, synthetic construct
  REGION 1..122: note = hu30VH7
EVRLQQSGPVVVKPGASVKVSCKASGYTFTDYYMNWVRQAPGQSLEWMGIINPYNGDTSYNQKFRGRVTLTVDKSASTAYMELSSLRSEDTAVYYCARYHYGPHLEGYFDVWGQGTTVTVSS

SEQ ID NO: 112 - protein, 122 aa, synthetic construct
  REGION 1..122: note = hu30VH8
EVRLVQFGAVVKKPGASVKVSCKASGYTFTDYYMNWVRQAPGQSLEWMGIINPYTGDTSYNQKFRGRVTLTVDKSSSTAYMELSSLRSEDTAVYYCARYHYGPHLEGYFDVWGQGTTVTVSS

SEQ ID NO: 113 - protein, 122 aa, synthetic construct
  REGION 1..122: note = hu30VH9
EVRLVQSGAEVKKPGASVKVSCKASGYTFTDYYMNWVRQAPGQSLEWIGIINPYTGDTSYNQKFRGRATLTVDKSASTAYMELSSLRSEDTAVYYCARYHYGPHLEGYFDVWGQGTTVTVSS

SEQ ID NO: 114 - protein, 122 aa, synthetic construct
  REGION 1..122: note = hu30VH10
EVRLVQSGAEVKKPGASVKVSCKASGYTFTDYYMNWVRQSHGQSLEWMGIINPYTGDTSYNQKFRGRVTLTVDKSASTAYMELSSLRSEDTAVYYCARYHYGPHLEGYFDVWGQGTTVTVSS

SEQ ID NO: 115 - protein, 122 aa, synthetic construct
  REGION 1..122: note = hu30VH11
EVRLVQFGAVVKKPGASVKVSCKASGYTFTDYYMNWVRQAPGQSLEWMGIINPYTGDTSYNQKFRGRVTLTVDKSSSTAYMELSSLTSEDTAVYYCARYHYGPHLEGYFDVWGQGTTVTVSS

SEQ ID NO: 116 - protein, 122 aa, synthetic construct
  REGION 1..122: note = hu30VH12
QVQLVQSGAEVKKPGASVKVSCKASGYTFTDYYMNWVRQAPGQRLEWMGIINPYNGDTSYNQKFRGRVTITRDTSASTAYMELSSLRSEDTAVYYCARYHYGPHLEGYFDVWGQGTTVTVSS

SEQ ID NO: 117 - protein, 17 aa, synthetic construct
  REGION 1..17: note = hu30VH3, HCDR2
IINPYQGDTSYNQKFRG

SEQ ID NO: 118 - protein, 17 aa, synthetic construct
  REGION 1..17: note = hu30VH4, HCDR2
IINPYSGDTSYNQKFRG

SEQ ID NO: 119 - protein, 17 aa, synthetic construct
  REGION 1..17: note = hu30VH5/VH8/VH9/VH10/VH11 HCDR2
IINPYTGDTSYNQKFRG

SEQ ID NO: 120 - protein, 17 aa, synthetic construct
  REGION 1..17: note = hu30VH6, HCDR2
IINPYNVDTSYNQKFRG

SEQ ID NO: 121 - protein, 450 aa, synthetic construct
  REGION 1..450: note = Hu6 hu6L4H12
EVQLVQSGSELKKPGASVKVSCKASGYTFTDYYMNWVRQAPGQGLEWMGIINPYSGVTIYNHKFKGRFALSVDKSSNTAYLQISSLKAEDTAVYYCARQDSLLDYAMDYWGQGTTVTVSSASTKGPSVFPLAPSSKSTSGGTAALGCLVKDYFPEPVTVSWNSGALTSGVHTFPAVLQSSGLYSLSSVVTVPSSSLGTQTYICNVNHKPSNTKVDKKVEPKSCDKTHTCPPCPAPELLGGPSVFLFPPKPKDTLMISRTPEVTCVVVDVSHEDPEVKFNWYVDGVEVHNAKTKPREEQYNSTYRVVSVLTVLHQDWLNGKEYKCKVSNKALPAPIEKTISKAKGQPREPQVYTLPPSRDELTKNQVSLTCLVKGFYPSDIAVEWESNGQPENNYKTTPPVLDSDGSFFLYSKLTVDKSRWQQGNVFSCSVMHEALHNHYTQKSLSLSPGK

SEQ ID NO: 122 - protein, 214 aa, synthetic construct
  REGION 1..214: note = Hu6 hu6L4H12
DIQMTQSPSSLSASVGDRVTITCHASQGISGNMGWLQQKPGKAPKGLIYHGANLEDGVPSRFSGSGSGADYTLTISSLQPEDFADYYCVQYAQFPYTFGGGTKVEIKRTVAAPSVFIFPPSDEQLKSGTASVVCLLNNFYPREAKVQWKVDNALQSGNSQESVTEQDSKDSTYSLSSTLTLSKADYEKHKVYACEVTHQGLSSPVTKSFNRGEC

SEQ ID NO: 123 - protein, 451 aa, synthetic construct
  REGION 1..451: note = Hu98 hu98L3H4
EVQLVESGGGLVQPGGSLRLSCAASGFTFSDYGIHWVRQAPGKGLEWVAYISSGGYTSYYADTVKGRFTISRDNAKNSLYLQMNSLRAEDTAVYYCARGDYEDIFYTMDYWGQGTTVTVSSASTKGPSVFPLAPSSKSTSGGTAALGCLVKDYFPEPVTVSWNSGALTSGVHTFPAVLQSSGLYSLSSVVTVPSSSLGTQTYICNVNHKPSNTKVDKKVEPKSCDKTHTCPPCPAPELLGGPSVFLFPPKPKDTLMISRTPEVTCVVVDVSHEDPEVKFNWYVDGVEVHNAKTKPREEQYNSTYRVVSVLTVLHQDWLNGKEYKCKVSNKALPAPIEKTISKAKGQPREPQVYTLPPSRDELTKNQVSLTCLVKGFYPSDIAVEWESNGQPENNYKTTPPVLDSDGSFFLYSKLTVDKSRWQQGNVFSCSVMHEALHNHYTQKSLSLSPGK

SEQ ID NO: 124 - protein, 214 aa, synthetic construct
  REGION 1..214: note = Hu98 hu98L3H4
DIQMTQSPSSLSASVGDRVTITCRASRDITKFLNWYQQKPGGAVKLLIYYTSRLHSGVPSRFSGSGSGTDYTLTISSLQPEDFATYYCQQGNTLPWTFGGGTKVEIKRTVAAPSVFIFPPSDEQLKSGTASVVCLLNNFYPREAKVQWKVDNALQSGNSQESVTEQDSKDSTYSLSSTLTLSKADYEKHKVYACEVTHQGLSSPVTKSFNRGEC

SEQ ID NO: 125 - protein, 454 aa, synthetic construct
  REGION 1..454: note = Hu110 hu110L2H3
EVQLVQSGAEVKKPGASVKVSCKTSGYTFTDYYMNWVRQAPGQSLEWMGIINPYQGGTSYTQKFKGRVTITVDKSASTAYMELSSLRSEDTAVYYCARHFYDSSYLTYSTMDYWGQGTTVTVSSASTKGPSVFPLAPSSKSTSGGTAALGCLVKDYFPEPVTVSWNSGALTSGVHTFPAVLQSSGLYSLSSVVTVPSSSLGTQTYICNVNHKPSNTKVDKKVEPKSCDKTHTCPPCPAPELLGGPSVFLFPPKPKDTLMISRTPEVTCVVVDVSHEDPEVKFNWYVDGVEVHNAKTKPREEQYNSTYRVVSVLTVLHQDWLNGKEYKCKVSNKALPAPIEKTISKAKGQPREPQVYTLPPSRDELTKNQVSLTCLVKGFYPSDIAVEWESNGQPENNYKTTPPVLDSDGSFFLYSKLTVDKSRWQQGNVFSCSVMHEALHNHYTQKSLSLSPGK

SEQ ID NO: 126 - protein, 214 aa, synthetic construct
  REGION 1..214: note = Hu110 hu110L2H3
NIVMTQSPKSLAVSLGERATINCKASENVGIFVSWYQQKPGQSPKLLIYGASNRYTGVPDRFSGSGSATDFTLTISSLQAEDVADYYCGQSHSYPLTFGQGTKLEIKRTVAAPSVFIFPPSDEQLKSGTASVVCLLNNFYPREAKVQWKVDNALQSGNSQESVTEQDSKDSTYSLSSTLTLSKADYEKHKVYACEVTHQGLSSPVTKSFNRGEC

SEQ ID NO: 127 - protein, 452 aa, synthetic construct
  REGION 1..452: note = Hu30 hu30L1H5
EVRLVQSGAEVKKPGASVKVSCKASGYTFTDYYMNWVRQAPGQSLEWMGIINPYTGDTSYNQKFRGRVTLTVDKSASTAYMELSSLRSEDTAVYYCARYHYGPHLEGYFDVWGQGTTVTVSSASTKGPSVFPLAPSSKSTSGGTAALGCLVKDYFPEPVTVSWNSGALTSGVHTFPAVLQSSGLYSLSSVVTVPSSSLGTQTYICNVNHKPSNTKVDKKVEPKSCDKTHTCPPCPAPELLGGPSVFLFPPKPKDTLMISRTPEVTCVVVDVSHEDPEVKFNWYVDGVEVHNAKTKPREEQYNSTYRVVSVLTVLHQDWLNGKEYKCKVSNKALPAPIEKTISKAKGQPREPQVYTLPPSRDELTKNQVSLTCLVKGFYPSDIAVEWESNGQPENNYKTTPPVLDSDGSFFLYSKLTVDKSRWQQGNVFSCSVMHEALHNHYTQKSLSLSPGK

SEQ ID NO: 128 - protein, 213 aa, synthetic construct
  REGION 1..213: note = Hu30 hu30L1H5
DIVMTQSPDSLAVSLGERATINCKASENVGYVSWYQQKPGQPPKLLIYGASNRYTGVPDRFSGSGSGTDFTLTISSLQAEDVAVYYCGQSYSYPLTFGQGTKLEIKRTVAAPSVFIFPPSDEQLKSGTASVVCLLNNFYPREAKVQWKVDNALQSGNSQESVTEQDSKDSTYSLSSTLTLSKADYEKHKVYACEVTHQGLSSPVTKSFNRGEC

SEQ ID NO: 129 - protein, 5 aa, synthetic construct
  REGION 1..5: note = S107E I2C HCDR1
KYAMN

SEQ ID NO: 130 - protein, 19 aa, synthetic construct
  REGION 1..19: note = S107E I2C HCDR2
RIRSKYNNYATYYADSVKD

SEQ ID NO: 131 - protein, 14 aa, synthetic construct
  REGION 1..14: note = S107E HCDR3
HGNFGNEYISYWAY

SEQ ID NO: 132 - protein, 14 aa, synthetic construct
  REGION 1..14: note = S107E I2C LCDR1
GSSTGAVTSGNYPN

SEQ ID NO: 133 - protein, 7 aa, synthetic construct
  REGION 1..7: note = S107E I2C LCDR2
GTKFLAP

SEQ ID NO: 134 - protein, 9 aa, synthetic construct
  REGION 1..9: note = S107E I2C LCDR3
VLWYSNRWV

SEQ ID NO: 135 - protein, 14 aa, synthetic construct
  REGION 1..14: note = I2C HCDR3
HGNFGNSYISYWAY

SEQ ID NO: 136 - protein, 125 aa, synthetic construct
  REGION 1..125: note = S107E-VH
EVQLVESGGGLVQPGGSLKLSCAASGFTFNKYAMNWVRQAPGKGLEWVARIRSKYNNYATYYADSVKDRFTISRDDSKNTAYLQMNNLKTEDTAVYYCVRHGNFGNEYISYWAYWGQGTLVTVSS

SEQ ID NO: 137 - protein, 109 aa, synthetic construct
  REGION 1..109: note = S107E IC2-VL
QTVVTQEPSLTVSPGGTVTLTCGSSTGAVTSGNYPNWVQQKPGQAPRGLIGGTKFLAPGTPARFSGSLLGGKAALTLSGVQPEDEAEYYCVLWYSNRWVFGGGTKLTVL

SEQ ID NO: 138 - protein, 125 aa, synthetic construct
  REGION 1..125: note = I2C-VH
EVQLVESGGGLVQPGGSLKLSCAASGFTFNKYAMNWVRQAPGKGLEWVARIRSKYNNYATYYADSVKDRFTISRDDSKNTAYLQMNNLKTEDTAVYYCVRHGNFGNSYISYWAYWGQGTLVTVSS

SEQ ID NO: 139 - protein, 249 aa, synthetic construct
  REGION 1..249: note = S107E-scFv
EVQLVESGGGLVQPGGSLKLSCAASGFTFNKYAMNWVRQAPGKGLEWVARIRSKYNNYATYYADSVKDRFTISRDDSKNTAYLQMNNLKTEDTAVYYCVRHGNFGNEYISYWAYWGQGTLVTVSSGGGGSGGGGSGGGGSQTVVTQEPSLTVSPGGTVTLTCGSSTGAVTSGNYPNWVQQKPGQAPRGLIGGTKFLAPGTPARFSGSLLGGKAALTLSGVQPEDEAEYYCVLWYSNRWVFGGGTKLTVL

SEQ ID NO: 140 - protein, 249 aa, synthetic construct
  REGION 1..249: note = I2C-scFv
EVQLVESGGGLVQPGGSLKLSCAASGFTFNKYAMNWVRQAPGKGLEWVARIRSKYNNYATYYADSVKDRFTISRDDSKNTAYLQMNNLKTEDTAVYYCVRHGNFGNSYISYWAYWGQGTLVTVSSGGGGSGGGGSGGGGSQTVVTQEPSLTVSPGGTVTLTCGSSTGAVTSGNYPNWVQQKPGQAPRGLIGGTKFLAPGTPARFSGSLLGGKAALTLSGVQPEDEAEYYCVLWYSNRWVFGGGTKLTVL

SEQ ID NO: 141 - protein, 103 aa, synthetic construct
  REGION 1..103: note = IgG1(CH1)
ASTKGPSVFPLAPSSKSTSGGTAALGCLVKDYFPEPVTVSWNSGALTSGVHTFPAVLQSSGLYSLSSVVTVPSSSLGTQTYICNVNHKPSNTKVDKKVEPKSC

SEQ ID NO: 142 - protein, 105 aa, synthetic construct
  REGION 1..105: note = h
GQPKANPTVTLFPPSSEELQANKATLVCLISDFYPGAVTVAWKADGSPVKAGVETTKPSKQSNNKYAASSYLSLTPEQWKSHRSYSCQVTHEGSTVEKTVAPTEC

SEQ ID NO: 143 - protein, 227 aa, synthetic construct
  REGION 1..227: note = IgG1Fc knob
DKTHTCPPCPAPEAAGGPSVFLFPPKPKDTLMISRTPEVTCVVVDVSHEDPEVKFNWYVDGVEVHNAKTKPREEQYNSTYRVVSVLTVLHQDWLNGKEYKCKVSNKALPAPIEKTISKAKGQPREPQVYTLPPCREEMTKNQVSLWCLVKGFYPSDIAVEWESNGQPENNYKTTPPVLDSDGSFFLYSKLTVDKSRWQQGNVFSCSVMHEALHNHYTQKSLSLSPGK

SEQ ID NO: 144 - protein, 227 aa, synthetic construct
  REGION 1..227: note = IgG1Fc hole
DKTHTCPPCPAPEAAGGPSVFLFPPKPKDTLMISRTPEVTCVVVDVSHEDPEVKFNWYVDGVEVHNAKTKPREEQYNSTYRVVSVLTVLHQDWLNGKEYKCKVSNKALPAPIEKTISKAKGQPREPQVCTLPPSREEMTKNQVSLSCAVKGFYPSDIAVEWESNGQPENNYKTTPPVLDSDGSFFLVSKLTVDKSRWQQGNVFSCSVMHEALHNHYTQKSLSLSPGK

SEQ ID NO: 145 - protein, 222 aa, synthetic construct
  REGION 1..222: note = Fc knob
CPPCPAPEAAGAPSVFLFPPKPKDTLMISRTPEVTCVVVDVSHEDPEVKFNWYVDGVEVHNAKTKPREEQYNSTYRVVSVLTVLHQDWLNGKEYKCKVSNKALPAPIEKTISKAKGQPREPQVCTLPPSREEMTKNQVSLWCLVKGFYPSDIAVEWESNGQPENNYKTTPPVLDSDGSFFLYSKLTVDKSRWQQGNVFSCSVMHEALHNHYTQKSLSLSPGK

SEQ ID NO: 146 - protein, 222 aa, synthetic construct
  REGION 1..222: note = Fc hole
CPPCPAPEAAGAPSVFLFPPKPKDTLMISRTPEVTCVVVDVSHEDPEVKFNWYVDGVEVHNAKTKPREEQYNSTYRVVSVLTVLHQDWLNGKEYKCKVSNKALPAPIEKTISKAKGQPREPQVYTLPPCREEMTKNQVSLSCAVKGFYPSDIAVEWESNGQPENNYKTTPPVLDSDGSFFLVSKLTVDKSRWQQGNVFSCSVMHEALHNHYTQKSLSLSPGK

SEQ ID NO: 147 - protein, 5 aa, synthetic construct
  REGION 1..5: note = Linker1
GGGGS

SEQ ID NO: 148 - protein, 15 aa, synthetic construct
  REGION 1..15: note = Linker2
GGGGSGGGGSGGGGS

SEQ ID NO: 149 - protein, 8 aa, synthetic construct
  REGION 1..8: note = Linke3
GGGSGGGG

SEQ ID NO: 150 - skipped

SEQ ID NO: 151 - protein, 9 aa, synthetic construct
  REGION 1..9: note = Linke5
GGGGSGGGG

SEQ ID NO: 152 - protein, 209 aa, synthetic construct
  REGION 1..209: note = hu6VL-G4S-Obscurin
DIQMTQSPSSLSASVGDRVTITCHASQGISGNMGWLQQKPGKAPKGLIYHGANLEDGVPSRFSGSGSGADYTLTISSLQPEDFADYYCVQYAQFPYTFGGGTKVEIKGGGGSSGAPRFLTRPKASVVSVGKDATLSCQIVGNPFPQVSWEKDKQPVTAGVRFRLAQDGDLYRLKILDLQLSDSGQYVCRARNAHGEAFACLGLQVDAEA

SEQ ID NO: 153 - protein, 450 aa, synthetic construct
  REGION 1..450: note = hu6VH-G4S-Titin-hole
EVQLVQSGSELKKPGASVKVSCKASGYTFTDYYMNWVRQAPGQGLEWMGIINPYSGVTIYNHKFKGRFALSVDKSSNTAYLQISSLKAEDTAVYYCARQDSLLDYAMDYWGQGTTVTVSSGGGGSGIPPKIECLPIDISIDEGKVLTVASAFTGEPTPEVTWSTGGRKIHSQEQGRFHIENTDDSTTLTIKDVQKQDGGLYTLTLRNEFGSDSATVNIHIRSIDKTHTCPPCPAPEAAGGPSVFLFPPKPKDTLMISRTPEVTCVVVDVSHEDPEVKFNWYVDGVEVHNAKTKPREEQYNSTYRVVSVLTVLHQDWLNGKEYKCKVSNKALPAPIEKTISKAKGQPREPQVCTLPPSREEMTKNQVSLSCAVKGFYPSDIAVEWESNGQPENNYKTTPPVLDSDGSFFLVSKLTVDKSRWQQGNVFSCSVMHEALHNHYTQKSLSLSPGK

SEQ ID NO: 154 - protein, 455 aa, synthetic construct
  REGION 1..455: note = S107EVH-CH1-knob
EVQLVESGGGLVQPGGSLKLSCAASGFTFNKYAMNWVRQAPGKGLEWVARIRSKYNNYATYYADSVKDRFTISRDDSKNTAYLQMNNLKTEDTAVYYCVRHGNFGNEYISYWAYWGQGTLVTVSSASTKGPSVFPLAPSSKSTSGGTAALGCLVKDYFPEPVTVSWNSGALTSGVHTFPAVLQSSGLYSLSSVVTVPSSSLGTQTYICNVNHKPSNTKVDKKVEPKSCDKTHTCPPCPAPEAAGGPSVFLFPPKPKDTLMISRTPEVTCVVVDVSHEDPEVKFNWYVDGVEVHNAKTKPREEQYNSTYRVVSVLTVLHQDWLNGKEYKCKVSNKALPAPIEKTISKAKGQPREPQVYTLPPCREEMTKNQVSLWCLVKGFYPSDIAVEWESNGQPENNYKTTPPVLDSDGSFFLYSKLTVDKSRWQQGNVFSCSVMHEALHNHYTQKSLSLSPGK

SEQ ID NO: 155 - protein, 214 aa, synthetic construct
  REGION 1..214: note = CD3VL-h
QTVVTQEPSLTVSPGGTVTLTCGSSTGAVTSGNYPNWVQQKPGQAPRGLIGGTKFLAPGTPARFSGSLLGGKAALTLSGVQPEDEAEYYCVLWYSNRWVFGGGTKLTVLGQPKANPTVTLFPPSSEELQANKATLVCLISDFYPGAVTVAWKADGSPVKAGVETTKPSKQSNNKYAASSYLSLTPEQWKSHRSYSCQVTHEGSTVEKTVAPTEC

SEQ ID NO: 156 - protein, 455 aa, synthetic construct
  REGION 1..455: note = I2CVH-CH1-knob
EVQLVESGGGLVQPGGSLKLSCAASGFTFNKYAMNWVRQAPGKGLEWVARIRSKYNNYATYYADSVKDRFTISRDDSKNTAYLQMNNLKTEDTAVYYCVRHGNFGNSYISYWAYWGQGTLVTVSSASTKGPSVFPLAPSSKSTSGGTAALGCLVKDYFPEPVTVSWNSGALTSGVHTFPAVLQSSGLYSLSSVVTVPSSSLGTQTYICNVNHKPSNTKVDKKVEPKSCDKTHTCPPCPAPEAAGGPSVFLFPPKPKDTLMISRTPEVTCVVVDVSHEDPEVKFNWYVDGVEVHNAKTKPREEQYNSTYRVVSVLTVLHQDWLNGKEYKCKVSNKALPAPIEKTISKAKGQPREPQVYTLPPCREEMTKNQVSLWCLVKGFYPSDIAVEWESNGQPENNYKTTPPVLDSDGSFFLYSKLTVDKSRWQQGNVFSCSVMHEALHNHYTQKSLSLSPGK

SEQ ID NO: 157 - protein, 214 aa, synthetic construct; identical to SEQ ID NO: 122
  REGION 1..214: note = hu6VL-h

SEQ ID NO: 158 - protein, 450 aa, synthetic construct
  REGION 1..450: note = hu6VH-CH1-hole
EVQLVQSGSELKKPGASVKVSCKASGYTFTDYYMNWVRQAPGQGLEWMGIINPYSGVTIYNHKFKGRFALSVDKSSNTAYLQISSLKAEDTAVYYCARQDSLLDYAMDYWGQGTTVTVSSASTKGPSVFPLAPSSKSTSGGTAALGCLVKDYFPEPVTVSWNSGALTSGVHTFPAVLQSSGLYSLSSVVTVPSSSLGTQTYICNVNHKPSNTKVDKKVEPKSCDKTHTCPPCPAPEAAGGPSVFLFPPKPKDTLMISRTPEVTCVVVDVSHEDPEVKFNWYVDGVEVHNAKTKPREEQYNSTYRVVSVLTVLHQDWLNGKEYKCKVSNKALPAPIEKTISKAKGQPREPQVCTLPPSREEMTKNQVSLSCAVKGFYPSDIAVEWESNGQPENNYKTTPPVLDSDGSFFLVSKLTVDKSRWQQGNVFSCSVMHEALHNHYTQKSLSLSPGK

SEQ ID NO: 159 - protein, 481 aa, synthetic construct
  REGION 1..481: note = S107E_scFv-knob
EVQLVESGGGLVQPGGSLKLSCAASGFTFNKYAMNWVRQAPGKGLEWVARIRSKYNNYATYYADSVKDRFTISRDDSKNTAYLQMNNLKTEDTAVYYCVRHGNFGNEYISYWAYWGQGTLVTVSSGGGGSGGGGSGGGGSQTVVTQEPSLTVSPGGTVTLTCGSSTGAVTSGNYPNWVQQKPGQAPRGLIGGTKFLAPGTPARFSGSLLGGKAALTLSGVQPEDEAEYYCVLWYSNRWVFGGGTKLTVLGGGGSDKTHTCPPCPAPEAAGGPSVFLFPPKPKDTLMISRTPEVTCVVVDVSHEDPEVKFNWYVDGVEVHNAKTKPREEQYNSTYRVVSVLTVLHQDWLNGKEYKCKVSNKALPAPIEKTISKAKGQPREPQVYTLPPCREEMTKNQVSLWCLVKGFYPSDIAVEWESNGQPENNYKTTPPVLDSDGSFFLYSKLTVDKSRWQQGNVFSCSVMHEALHNHYTQKSLSLSPGK

SEQ ID NO: 160 - protein, 481 aa, synthetic construct
  REGION 1..481: note = I2C_scFv-knob
EVQLVESGGGLVQPGGSLKLSCAASGFTFNKYAMNWVRQAPGKGLEWVARIRSKYNNYATYYADSVKDRFTISRDDSKNTAYLQMNNLKTEDTAVYYCVRHGNFGNSYISYWAYWGQGTLVTVSSGGGGSGGGGSGGGGSQTVVTQEPSLTVSPGGTVTLTCGSSTGAVTSGNYPNWVQQKPGQAPRGLIGGTKFLAPGTPARFSGSLLGGKAALTLSGVQPEDEAEYYCVLWYSNRWVFGGGTKLTVLGGGGSDKTHTCPPCPAPEAAGGPSVFLFPPKPKDTLMISRTPEVTCVVVDVSHEDPEVKFNWYVDGVEVHNAKTKPREEQYNSTYRVVSVLTVLHQDWLNGKEYKCKVSNKALPAPIEKTISKAKGQPREPQVYTLPPCREEMTKNQVSLWCLVKGFYPSDIAVEWESNGQPENNYKTTPPVLDSDGSFFLYSKLTVDKSRWQQGNVFSCSVMHEALHNHYTQKSLSLSPGK

SEQ ID NO: 161 - protein, 463 aa, synthetic construct
  REGION 1..463: note = hu6VL-S107EVH-knob
DIQMTQSPSSLSASVGDRVTITCHASQGISGNMGWLQQKPGKAPKGLIYHGANLEDGVPSRFSGSGSGADYTLTISSLQPEDFADYYCVQYAQFPYTFGGGTKVEIKGGGSGGGGEVQLVESGGGLVQPGGSLKLSCAASGFTFNKYAMNWVRQAPGKGLEWVARIRSKYNNYATYYADSVKDRFTISRDDSKNTAYLQMNNLKTEDTAVYYCVRHGNFGNEYISYWAYWGQGTLVTVSSGCPPCPAPEAAGAPSVFLFPPKPKDTLMISRTPEVTCVVVDVSHEDPEVKFNWYVDGVEVHNAKTKPREEQYNSTYRVVSVLTVLHQDWLNGKEYKCKVSNKALPAPIEKTISKAKGQPREPQVCTLPPSREEMTKNQVSLWCLVKGFYPSDIAVEWESNGQPENNYKTTPPVLDSDGSFFLYSKLTVDKSRWQQGNVFSCSVMHEALHNHYTQKSLSLSPGK

SEQ ID NO: 162 - protein, 461 aa, synthetic construct
  REGION 1..461: note = CD3VL-hu6VH-hole
QTVVTQEPSLTVSPGGTVTLTCGSSTGAVTSGNYPNWVQQKPGQAPRGLIGGTKFLAPGTPARFSGSLLGGKAALTLSGVQPEDEAEYYCVLWYSNRWVFGGGTKLTVLGGGGSGGGGEVQLVQSGSELKKPGASVKVSCKASGYTFTDYYMNWVRQAPGQGLEWMGIINPYSGVTIYNHKFKGRFALSVDKSSNTAYLQISSLKAEDTAVYYCARQDSLLDYAMDYWGQGTTVTVSSGCPPCPAPEAAGAPSVFLFPPKPKDTLMISRTPEVTCVVVDVSHEDPEVKFNWYVDGVEVHNAKTKPREEQYNSTYRVVSVLTVLHQDWLNGKEYKCKVSNKALPAPIEKTISKAKGQPREPQVYTLPPCREEMTKNQVSLSCAVKGFYPSDIAVEWESNGQPENNYKTTPPVLDSDGSFFLVSKLTVDKSRWQQGNVFSCSVMHEALHNHYTQKSLSLSPGK

SEQ ID NO: 163 - protein, 463 aa, synthetic construct
  REGION 1..463: note = hu6VL-I2CVH-knob
DIQMTQSPSSLSASVGDRVTITCHASQGISGNMGWLQQKPGKAPKGLIYHGANLEDGVPSRFSGSGSGADYTLTISSLQPEDFADYYCVQYAQFPYTFGGGTKVEIKGGGSGGGGEVQLVESGGGLVQPGGSLKLSCAASGFTFNKYAMNWVRQAPGKGLEWVARIRSKYNNYATYYADSVKDRFTISRDDSKNTAYLQMNNLKTEDTAVYYCVRHGNFGNSYISYWAYWGQGTLVTVSSGCPPCPAPEAAGAPSVFLFPPKPKDTLMISRTPEVTCVVVDVSHEDPEVKFNWYVDGVEVHNAKTKPREEQYNSTYRVVSVLTVLHQDWLNGKEYKCKVSNKALPAPIEKTISKAKGQPREPQVCTLPPSREEMTKNQVSLWCLVKGFYPSDIAVEWESNGQPENNYKTTPPVLDSDGSFFLYSKLTVDKSRWQQGNVFSCSVMHEALHNHYTQKSLSLSPGK

SEQ ID NO: 164 - protein, 209 aa, synthetic construct
  REGION 1..209: note = hu98VL-G4S-Obscurin
DIQMTQSPSSLSASVGDRVTITCRASRDITKFLNWYQQKPGGAVKLLIYYTSRLHSGVPSRFSGSGSGTDYTLTISSLQPEDFATYYCQQGNTLPWTFGGGTKVEIKGGGGSSGAPRFLTRPKASVVSVGKDATLSCQIVGNPFPQVSWEKDKQPVTAGVRFRLAQDGDLYRLKILDLQLSDSGQYVCRARNAHGEAFACLGLQVDAEA

SEQ ID NO: 165 - protein, 451 aa, synthetic construct
  REGION 1..451: note = hu98VH-G4S-Titin-hole
EVQLVESGGGLVQPGGSLRLSCAASGFTFSDYGIHWVRQAPGKGLEWVAYISSGGYTSYYADTVKGRFTISRDNAKNSLYLQMNSLRAEDTAVYYCARGDYEDIFYTMDYWGQGTTVTVSSGGGGSGIPPKIECLPIDISIDEGKVLTVASAFTGEPTPEVTWSTGGRKIHSQEQGRFHIENTDDSTTLTIKDVQKQDGGLYTLTLRNEFGSDSATVNIHIRSIDKTHTCPPCPAPEAAGGPSVFLFPPKPKDTLMISRTPEVTCVVVDVSHEDPEVKFNWYVDGVEVHNAKTKPREEQYNSTYRVVSVLTVLHQDWLNGKEYKCKVSNKALPAPIEKTISKAKGQPREPQVCTLPPSREEMTKNQVSLSCAVKGFYPSDIAVEWESNGQPENNYKTTPPVLDSDGSFFLVSKLTVDKSRWQQGNVFSCSVMHEALHNHYTQKSLSLSPGK

SEQ ID NO: 166 - protein, 214 aa, synthetic construct; identical to SEQ ID NO: 124
  REGION 1..214: note = hu98VL-h

SEQ ID NO: 167 - protein, 451 aa, synthetic construct
  REGION 1..451: note = hu98VH-CH1-hole
EVQLVESGGGLVQPGGSLRLSCAASGFTFSDYGIHWVRQAPGKGLEWVAYISSGGYTSYYADTVKGRFTISRDNAKNSLYLQMNSLRAEDTAVYYCARGDYEDIFYTMDYWGQGTTVTVSSASTKGPSVFPLAPSSKSTSGGTAALGCLVKDYFPEPVTVSWNSGALTSGVHTFPAVLQSSGLYSLSSVVTVPSSSLGTQTYICNVNHKPSNTKVDKKVEPKSCDKTHTCPPCPAPEAAGGPSVFLFPPKPKDTLMISRTPEVTCVVVDVSHEDPEVKFNWYVDGVEVHNAKTKPREEQYNSTYRVVSVLTVLHQDWLNGKEYKCKVSNKALPAPIEKTISKAKGQPREPQVCTLPPSREEMTKNQVSLSCAVKGFYPSDIAVEWESNGQPENNYKTTPPVLDSDGSFFLVSKLTVDKSRWQQGNVFSCSVMHEALHNHYTQKSLSLSPGK

SEQ ID NO: 168 - protein, 463 aa, synthetic construct
  REGION 1..463: note = hu98VL-S107EVH-knob
DIQMTQSPSSLSASVGDRVTITCRASRDITKFLNWYQQKPGGAVKLLIYYTSRLHSGVPSRFSGSGSGTDYTLTISSLQPEDFATYYCQQGNTLPWTFGGGTKVEIKGGGSGGGGEVQLVESGGGLVQPGGSLKLSCAASGFTFNKYAMNWVRQAPGKGLEWVARIRSKYNNYATYYADSVKDRFTISRDDSKNTAYLQMNNLKTEDTAVYYCVRHGNFGNEYISYWAYWGQGTLVTVSSGCPPCPAPEAAGAPSVFLFPPKPKDTLMISRTPEVTCVVVDVSHEDPEVKFNWYVDGVEVHNAKTKPREEQYNSTYRVVSVLTVLHQDWLNGKEYKCKVSNKALPAPIEKTISKAKGQPREPQVCTLPPSREEMTKNQVSLWCLVKGFYPSDIAVEWESNGQPENNYKTTPPVLDSDGSFFLYSKLTVDKSRWQQGNVFSCSVMHEALHNHYTQKSLSLSPGK

SEQ ID NO: 169 - protein, 462 aa, synthetic construct
  REGION 1..462: note = CD3VL-hu98VH-hole
QTVVTQEPSLTVSPGGTVTLTCGSSTGAVTSGNYPNWVQQKPGQAPRGLIGGTKFLAPGTPARFSGSLLGGKAALTLSGVQPEDEAEYYCVLWYSNRWVFGGGTKLTVLGGGGSGGGGEVQLVESGGGLVQPGGSLRLSCAASGFTFSDYGIHWVRQAPGKGLEWVAYISSGGYTSYYADTVKGRFTISRDNAKNSLYLQMNSLRAEDTAVYYCARGDYEDIFYTMDYWGQGTTVTVSSGCPPCPAPEAAGAPSVFLFPPKPKDTLMISRTPEVTCVVVDVSHEDPEVKFNWYVDGVEVHNAKTKPREEQYNSTYRVVSVLTVLHQDWLNGKEYKCKVSNKALPAPIEKTISKAKGQPREPQVYTLPPCREEMTKNQVSLSCAVKGFYPSDIAVEWESNGQPENNYKTTPPVLDSDGSFFLVSKLTVDKSRWQQGNVFSCSVMHEALHNHYTQKSLSLSPGK

SEQ ID NO: 170 - protein, 463 aa, synthetic construct
  REGION 1..463: note = hu98VL-I2CVH-knob
DIQMTQSPSSLSASVGDRVTITCRASRDITKFLNWYQQKPGGAVKLLIYYTSRLHSGVPSRFSGSGSGTDYTLTISSLQPEDFATYYCQQGNTLPWTFGGGTKVEIKGGGSGGGGEVQLVESGGGLVQPGGSLKLSCAASGFTFNKYAMNWVRQAPGKGLEWVARIRSKYNNYATYYADSVKDRFTISRDDSKNTAYLQMNNLKTEDTAVYYCVRHGNFGNSYISYWAYWGQGTLVTVSSGCPPCPAPEAAGAPSVFLFPPKPKDTLMISRTPEVTCVVVDVSHEDPEVKFNWYVDGVEVHNAKTKPREEQYNSTYRVVSVLTVLHQDWLNGKEYKCKVSNKALPAPIEKTISKAKGQPREPQVCTLPPSREEMTKNQVSLWCLVKGFYPSDIAVEWESNGQPENNYKTTPPVLDSDGSFFLYSKLTVDKSRWQQGNVFSCSVMHEALHNHYTQKSLSLSPGK

SEQ ID NO: 171 - protein, 209 aa, synthetic construct
  REGION 1..209: note = hu110VL-G4S-Obscurin
NIVMTQSPKSLAVSLGERATINCKASENVGIFVSWYQQKPGQSPKLLIYGASNRYTGVPDRFSGSGSATDFTLTISSLQAEDVADYYCGQSHSYPLTFGQGTKLEIKGGGGSSGAPRFLTRPKASVVSVGKDATLSCQIVGNPFPQVSWEKDKQPVTAGVRFRLAQDGDLYRLKILDLQLSDSGQYVCRARNAHGEAFACLGLQVDAEA

SEQ ID NO: 172 - protein, 454 aa, synthetic construct
  REGION 1..454: note = hu110VH-G4S-Titin-hole
EVQLVQSGAEVKKPGASVKVSCKTSGYTFTDYYMNWVRQAPGQSLEWMGIINPYQGGTSYTQKFKGRVTITVDKSASTAYMELSSLRSEDTAVYYCARHFYDSSYLTYSTMDYWGQGTTVTVSSGGGGSGIPPKIECLPIDISIDEGKVLTVASAFTGEPTPEVTWSTGGRKIHSQEQGRFHIENTDDSTTLTIKDVQKQDGGLYTLTLRNEFGSDSATVNIHIRSIDKTHTCPPCPAPEAAGGPSVFLFPPKPKDTLMISRTPEVTCVVVDVSHEDPEVKFNWYVDGVEVHNAKTKPREEQYNSTYRVVSVLTVLHQDWLNGKEYKCKVSNKALPAPIEKTISKAKGQPREPQVCTLPPSREEMTKNQVSLSCAVKGFYPSDIAVEWESNGQPENNYKTTPPVLDSDGSFFLVSKLTVDKSRWQQGNVFSCSVMHEALHNHYTQKSLSLSPGK

SEQ ID NO: 173 - protein, 214 aa, synthetic construct; identical to SEQ ID NO: 126
  REGION 1..214: note = hu110VL-h

SEQ ID NO: 174 - protein, 454 aa, synthetic construct
  REGION 1..454: note = hu110VH-CH1-hole
EVQLVQSGAEVKKPGASVKVSCKTSGYTFTDYYMNWVRQAPGQSLEWMGIINPYQGGTSYTQKFKGRVTITVDKSASTAYMELSSLRSEDTAVYYCARHFYDSSYLTYSTMDYWGQGTTVTVSSASTKGPSVFPLAPSSKSTSGGTAALGCLVKDYFPEPVTVSWNSGALTSGVHTFPAVLQSSGLYSLSSVVTVPSSSLGTQTYICNVNHKPSNTKVDKKVEPKSCDKTHTCPPCPAPEAAGGPSVFLFPPKPKDTLMISRTPEVTCVVVDVSHEDPEVKFNWYVDGVEVHNAKTKPREEQYNSTYRVVSVLTVLHQDWLNGKEYKCKVSNKALPAPIEKTISKAKGQPREPQVCTLPPSREEMTKNQVSLSCAVKGFYPSDIAVEWESNGQPENNYKTTPPVLDSDGSFFLVSKLTVDKSRWQQGNVFSCSVMHEALHNHYTQKSLSLSPGK

SEQ ID NO: 175 - protein, 463 aa, synthetic construct
  REGION 1..463: note = hu110VL-S107EVH-knob
NIVMTQSPKSLAVSLGERATINCKASENVGIFVSWYQQKPGQSPKLLIYGASNRYTGVPDRFSGSGSATDFTLTISSLQAEDVADYYCGQSHSYPLTFGQGTKLEIKGGGSGGGGEVQLVESGGGLVQPGGSLKLSCAASGFTFNKYAMNWVRQAPGKGLEWVARIRSKYNNYATYYADSVKDRFTISRDDSKNTAYLQMNNLKTEDTAVYYCVRHGNFGNEYISYWAYWGQGTLVTVSSGCPPCPAPEAAGAPSVFLFPPKPKDTLMISRTPEVTCVVVDVSHEDPEVKFNWYVDGVEVHNAKTKPREEQYNSTYRVVSVLTVLHQDWLNGKEYKCKVSNKALPAPIEKTISKAKGQPREPQVCTLPPSREEMTKNQVSLWCLVKGFYPSDIAVEWESNGQPENNYKTTPPVLDSDGSFFLYSKLTVDKSRWQQGNVFSCSVMHEALHNHYTQKSLSLSPGK

SEQ ID NO: 176 - protein, 465 aa, synthetic construct
  REGION 1..465: note = CD3VL-hu110VH-hole
QTVVTQEPSLTVSPGGTVTLTCGSSTGAVTSGNYPNWVQQKPGQAPRGLIGGTKFLAPGTPARFSGSLLGGKAALTLSGVQPEDEAEYYCVLWYSNRWVFGGGTKLTVLGGGGSGGGGEVQLVQSGAEVKKPGASVKVSCKTSGYTFTDYYMNWVRQAPGQSLEWMGIINPYQGGTSYTQKFKGRVTITVDKSASTAYMELSSLRSEDTAVYYCARHFYDSSYLTYSTMDYWGQGTTVTVSSGCPPCPAPEAAGAPSVFLFPPKPKDTLMISRTPEVTCVVVDVSHEDPEVKFNWYVDGVEVHNAKTKPREEQYNSTYRVVSVLTVLHQDWLNGKEYKCKVSNKALPAPIEKTISKAKGQPREPQVYTLPPCREEMTKNQVSLSCAVKGFYPSDIAVEWESNGQPENNYKTTPPVLDSDGSFFLVSKLTVDKSRWQQGNVFSCSVMHEALHNHYTQKSLSLSPGK

SEQ ID NO: 177 - protein, 463 aa, synthetic construct
  REGION 1..463: note = hu110VL-I2CVH-knob
NIVMTQSPKSLAVSLGERATINCKASENVGIFVSWYQQKPGQSPKLLIYGASNRYTGVPDRFSGSGSATDFTLTISSLQAEDVADYYCGQSHSYPLTFGQGTKLEIKGGGSGGGGEVQLVESGGGLVQPGGSLKLSCAASGFTFNKYAMNWVRQAPGKGLEWVARIRSKYNNYATYYADSVKDRFTISRDDSKNTAYLQMNNLKTEDTAVYYCVRHGNFGNSYISYWAYWGQGTLVTVSSGCPPCPAPEAAGAPSVFLFPPKPKDTLMISRTPEVTCVVVDVSHEDPEVKFNWYVDGVEVHNAKTKPREEQYNSTYRVVSVLTVLHQDWLNGKEYKCKVSNKALPAPIEKTISKAKGQPREPQVCTLPPSREEMTKNQVSLWCLVKGFYPSDIAVEWESNGQPENNYKTTPPVLDSDGSFFLYSKLTVDKSRWQQGNVFSCSVMHEALHNHYTQKSLSLSPGK

SEQ ID NO: 178 - protein, 208 aa, synthetic construct
  REGION 1..208: note = hu30VL-G4S-Obscurin
DIVMTQSPDSLAVSLGERATINCKASENVGYVSWYQQKPGQPPKLLIYGASNRYTGVPDRFSGSGSGTDFTLTISSLQAEDVAVYYCGQSYSYPLTFGQGTKLEIKGGGGSSGAPRFLTRPKASVVSVGKDATLSCQIVGNPFPQVSWEKDKQPVTAGVRFRLAQDGDLYRLKILDLQLSDSGQYVCRARNAHGEAFACLGLQVDAEA

SEQ ID NO: 179 - protein, 452 aa, synthetic construct
  REGION 1..452: note = hu30VH-G4S-Titin-hole
EVRLVQSGAEVKKPGASVKVSCKASGYTFTDYYMNWVRQAPGQSLEWMGIINPYTGDTSYNQKFRGRVTLTVDKSASTAYMELSSLRSEDTAVYYCARYHYGPHLEGYFDVWGQGTTVTVSSGGGGSGIPPKIECLPIDISIDEGKVLTVASAFTGEPTPEVTWSTGGRKIHSQEQGRFHIENTDDSTTLTIKDVQKQDGGLYTLTLRNEFGSDSATVNIHIRSIDKTHTCPPCPAPEAAGGPSVFLFPPKPKDTLMISRTPEVTCVVVDVSHEDPEVKFNWYVDGVEVHNAKTKPREEQYNSTYRVVSVLTVLHQDWLNGKEYKCKVSNKALPAPIEKTISKAKGQPREPQVCTLPPSREEMTKNQVSLSCAVKGFYPSDIAVEWESNGQPENNYKTTPPVLDSDGSFFLVSKLTVDKSRWQQGNVFSCSVMHEALHNHYTQKSLSLSPGK

SEQ ID NO: 180 - protein, 213 aa, synthetic construct; identical to SEQ ID NO: 128
  REGION 1..213: note = hu30VL-h

SEQ ID NO: 181 - protein, 452 aa, synthetic construct
  REGION 1..452: note = hu30VH-CH1-hole
EVRLVQSGAEVKKPGASVKVSCKASGYTFTDYYMNWVRQAPGQSLEWMGIINPYTGDTSYNQKFRGRVTLTVDKSASTAYMELSSLRSEDTAVYYCARYHYGPHLEGYFDVWGQGTTVTVSSASTKGPSVFPLAPSSKSTSGGTAALGCLVKDYFPEPVTVSWNSGALTSGVHTFPAVLQSSGLYSLSSVVTVPSSSLGTQTYICNVNHKPSNTKVDKKVEPKSCDKTHTCPPCPAPEAAGGPSVFLFPPKPKDTLMISRTPEVTCVVVDVSHEDPEVKFNWYVDGVEVHNAKTKPREEQYNSTYRVVSVLTVLHQDWLNGKEYKCKVSNKALPAPIEKTISKAKGQPREPQVCTLPPSREEMTKNQVSLSCAVKGFYPSDIAVEWESNGQPENNYKTTPPVLDSDGSFFLVSKLTVDKSRWQQGNVFSCSVMHEALHNHYTQKSLSLSPGK

SEQ ID NO: 182 - protein, 462 aa, synthetic construct
  REGION 1..462: note = hu30VL-S107EVH-knob
DIVMTQSPDSLAVSLGERATINCKASENVGYVSWYQQKPGQPPKLLIYGASNRYTGVPDRFSGSGSGTDFTLTISSLQAEDVAVYYCGQSYSYPLTFGQGTKLEIKGGGSGGGGEVQLVESGGGLVQPGGSLKLSCAASGFTFNKYAMNWVRQAPGKGLEWVARIRSKYNNYATYYADSVKDRFTISRDDSKNTAYLQMNNLKTEDTAVYYCVRHGNFGNEYISYWAYWGQGTLVTVSSGCPPCPAPEAAGAPSVFLFPPKPKDTLMISRTPEVTCVVVDVSHEDPEVKFNWYVDGVEVHNAKTKPREEQYNSTYRVVSVLTVLHQDWLNGKEYKCKVSNKALPAPIEKTISKAKGQPREPQVCTLPPSREEMTKNQVSLWCLVKGFYPSDIAVEWESNGQPENNYKTTPPVLDSDGSFFLYSKLTVDKSRWQQGNVFSCSVMHEALHNHYTQKSLSLSPGK

SEQ ID NO: 183 - protein, 463 aa, synthetic construct
  REGION 1..463: note = CD3VL-hu30VH-hole
QTVVTQEPSLTVSPGGTVTLTCGSSTGAVTSGNYPNWVQQKPGQAPRGLIGGTKFLAPGTPARFSGSLLGGKAALTLSGVQPEDEAEYYCVLWYSNRWVFGGGTKLTVLGGGGSGGGGEVRLVQSGAEVKKPGASVKVSCKASGYTFTDYYMNWVRQAPGQSLEWMGIINPYTGDTSYNQKFRGRVTLTVDKSASTAYMELSSLRSEDTAVYYCARYHYGPHLEGYFDVWGQGTTVTVSSGCPPCPAPEAAGAPSVFLFPPKPKDTLMISRTPEVTCVVVDVSHEDPEVKFNWYVDGVEVHNAKTKPREEQYNSTYRVVSVLTVLHQDWLNGKEYKCKVSNKALPAPIEKTISKAKGQPREPQVYTLPPCREEMTKNQVSLSCAVKGFYPSDIAVEWESNGQPENNYKTTPPVLDSDGSFFLVSKLTVDKSRWQQGNVFSCSVMHEALHNHYTQKSLSLSPGK

SEQ ID NO: 184 - protein, 462 aa, synthetic construct
  REGION 1..462: note = hu30VL-I2CVH-knob
DIVMTQSPDSLAVSLGERATINCKASENVGYVSWYQQKPGQPPKLLIYGASNRYTGVPDRFSGSGSGTDFTLTISSLQAEDVAVYYCGQSYSYPLTFGQGTKLEIKGGGSGGGGEVQLVESGGGLVQPGGSLKLSCAASGFTFNKYAMNWVRQAPGKGLEWVARIRSKYNNYATYYADSVKDRFTISRDDSKNTAYLQMNNLKTEDTAVYYCVRHGNFGNSYISYWAYWGQGTLVTVSSGCPPCPAPEAAGAPSVFLFPPKPKDTLMISRTPEVTCVVVDVSHEDPEVKFNWYVDGVEVHNAKTKPREEQYNSTYRVVSVLTVLHQDWLNGKEYKCKVSNKALPAPIEKTISKAKGQPREPQVCTLPPSREEMTKNQVSLWCLVKGFYPSDIAVEWESNGQPENNYKTTPPVLDSDGSFFLYSKLTVDKSRWQQGNVFSCSVMHEALHNHYTQKSLSLSPGK

SEQ ID NO: 185 - protein, 463 aa, synthetic construct
  REGION 1..463: note = hu6VL (D56E) -S107EVH-knob
DIQMTQSPSSLSASVGDRVTITCHASQGISGNMGWLQQKPGKAPKGLIYHGANLEEGVPSRFSGSGSGADYTLTISSLQPEDFADYYCVQYAQFPYTFGGGTKVEIKGGGSGGGGEVQLVESGGGLVQPGGSLKLSCAASGFTFNKYAMNWVRQAPGKGLEWVARIRSKYNNYATYYADSVKDRFTISRDDSKNTAYLQMNNLKTEDTAVYYCVRHGNFGNEYISYWAYWGQGTLVTVSSGCPPCPAPEAAGAPSVFLFPPKPKDTLMISRTPEVTCVVVDVSHEDPEVKFNWYVDGVEVHNAKTKPREEQYNSTYRVVSVLTVLHQDWLNGKEYKCKVSNKALPAPIEKTISKAKGQPREPQVCTLPPSREEMTKNQVSLWCLVKGFYPSDIAVEWESNGQPENNYKTTPPVLDSDGSFFLYSKLTVDKSRWQQGNVFSCSVMHEALHNHYTQKSLSLSPGK

SEQ ID NO: 186 - protein, 463 aa, synthetic construct
  REGION 1..463: note = hu6VL(D56S) -S107EVH-knob
DIQMTQSPSSLSASVGDRVTITCHASQGISGNMGWLQQKPGKAPKGLIYHGANLESGVPSRFSGSGSGADYTLTISSLQPEDFADYYCVQYAQFPYTFGGGTKVEIKGGGSGGGGEVQLVESGGGLVQPGGSLKLSCAASGFTFNKYAMNWVRQAPGKGLEWVARIRSKYNNYATYYADSVKDRFTISRDDSKNTAYLQMNNLKTEDTAVYYCVRHGNFGNEYISYWAYWGQGTLVTVSSGCPPCPAPEAAGAPSVFLFPPKPKDTLMISRTPEVTCVVVDVSHEDPEVKFNWYVDGVEVHNAKTKPREEQYNSTYRVVSVLTVLHQDWLNGKEYKCKVSNKALPAPIEKTISKAKGQPREPQVCTLPPSREEMTKNQVSLWCLVKGFYPSDIAVEWESNGQPENNYKTTPPVLDSDGSFFLYSKLTVDKSRWQQGNVFSCSVMHEALHNHYTQKSLSLSPGK

SEQ ID NO: 187 - protein, 463 aa, synthetic construct
  REGION 1..463: note = hu6VL8 -S107EVH-knob
DIQMTQSPSSLSASVGDRVTITCHASQGISGNMGWLQQKPGKAPKGLIYHGANLEEGVPSRFSGSGSGADYTLTISSLQPEDFADYYCVQYAQYPYTFGGGTKVEIKGGGSGGGGEVQLVESGGGLVQPGGSLKLSCAASGFTFNKYAMNWVRQAPGKGLEWVARIRSKYNNYATYYADSVKDRFTISRDDSKNTAYLQMNNLKTEDTAVYYCVRHGNFGNEYISYWAYWGQGTLVTVSSGCPPCPAPEAAGAPSVFLFPPKPKDTLMISRTPEVTCVVVDVSHEDPEVKFNWYVDGVEVHNAKTKPREEQYNSTYRVVSVLTVLHQDWLNGKEYKCKVSNKALPAPIEKTISKAKGQPREPQVCTLPPSREEMTKNQVSLWCLVKGFYPSDIAVEWESNGQPENNYKTTPPVLDSDGSFFLYSKLTVDKSRWQQGNVFSCSVMHEALHNHYTQKSLSLSPGK

SEQ ID NO: 188 - protein, 461 aa, synthetic construct
  REGION 1..461: note = CD3VL-hu6VH14-hole
QTVVTQEPSLTVSPGGTVTLTCGSSTGAVTSGNYPNWVQQKPGQAPRGLIGGTKFLAPGTPARFSGSLLGGKAALTLSGVQPEDEAEYYCVLWYSNRWVFGGGTKLTVLGGGGSGGGGEVQLVQSGSELKKPGASVKVSCKASGYTFTDYYMNWVRQAPGQGLEWMGIINPYSGVTTYNHKFKGRFALSVDKSSNTAYLQISSLKAEDTAVYYCARQDSLLDYAMDYWGQGTTVTVSSGCPPCPAPEAAGAPSVFLFPPKPKDTLMISRTPEVTCVVVDVSHEDPEVKFNWYVDGVEVHNAKTKPREEQYNSTYRVVSVLTVLHQDWLNGKEYKCKVSNKALPAPIEKTISKAKGQPREPQVYTLPPCREEMTKNQVSLSCAVKGFYPSDIAVEWESNGQPENNYKTTPPVLDSDGSFFLVSKLTVDKSRWQQGNVFSCSVMHEALHNHYTQKSLSLSPGK

SEQ ID NO: 189 - protein, 461 aa, synthetic construct
  REGION 1..461: note = CD3VL-hu6VH15-hole
QTVVTQEPSLTVSPGGTVTLTCGSSTGAVTSGNYPNWVQQKPGQAPRGLIGGTKFLAPGTPARFSGSLLGGKAALTLSGVQPEDEAEYYCVLWYSNRWVFGGGTKLTVLGGGGSGGGGEVQLQQSGSELKKPGASVKVSCKASGYTFTDYYMNWVRQAPGQGLEWMGIINPYSGSTIYNHKFKGRFALSVDKSSNTAYLQISSLKAEDTAVYYCARQDSLLDYAMDYWGQGTTVTVSSGCPPCPAPEAAGAPSVFLFPPKPKDTLMISRTPEVTCVVVDVSHEDPEVKFNWYVDGVEVHNAKTKPREEQYNSTYRVVSVLTVLHQDWLNGKEYKCKVSNKALPAPIEKTISKAKGQPREPQVYTLPPCREEMTKNQVSLSCAVKGFYPSDIAVEWESNGQPENNYKTTPPVLDSDGSFFLVSKLTVDKSRWQQGNVFSCSVMHEALHNHYTQKSLSLSPGK

SEQ ID NO: 190 - protein, 463 aa, synthetic construct
  REGION 1..463: note = hu6VL9-S107EVH-knob
NIQMTQSPSSLSASVGDRVTITCHASQGISGNMGWLQQKPGKAPKGLIYHGRNLEEGVPSRFSGSGSGADYTLTISSLQPEDFADYYCVQYAQYPYTFGGGTKVEIKGGGSGGGGEVQLVESGGGLVQPGGSLKLSCAASGFTFNKYAMNWVRQAPGKGLEWVARIRSKYNNYATYYADSVKDRFTISRDDSKNTAYLQMNNLKTEDTAVYYCVRHGNFGNEYISYWAYWGQGTLVTVSSGCPPCPAPEAAGAPSVFLFPPKPKDTLMISRTPEVTCVVVDVSHEDPEVKFNWYVDGVEVHNAKTKPREEQYNSTYRVVSVLTVLHQDWLNGKEYKCKVSNKALPAPIEKTISKAKGQPREPQVCTLPPSREEMTKNQVSLWCLVKGFYPSDIAVEWESNGQPENNYKTTPPVLDSDGSFFLYSKLTVDKSRWQQGNVFSCSVMHEALHNHYTQKSLSLSPGK

SEQ ID NO: 191 - protein, 463 aa, synthetic construct
  REGION 1..463: note = hu6VL10-S107EVH-knob
EIVLTQSPATLSLSPGERATLSCHASQGISGNMGWLQQKPGKAPRGLIYHGANLEEGIPARFSGSGSGADYTLTISRLQPEDFADYYCVQYAQFPYTFGGGTKVEIKGGGSGGGGEVQLVESGGGLVQPGGSLKLSCAASGFTFNKYAMNWVRQAPGKGLEWVARIRSKYNNYATYYADSVKDRFTISRDDSKNTAYLQMNNLKTEDTAVYYCVRHGNFGNEYISYWAYWGQGTLVTVSSGCPPCPAPEAAGAPSVFLFPPKPKDTLMISRTPEVTCVVVDVSHEDPEVKFNWYVDGVEVHNAKTKPREEQYNSTYRVVSVLTVLHQDWLNGKEYKCKVSNKALPAPIEKTISKAKGQPREPQVCTLPPSREEMTKNQVSLWCLVKGFYPSDIAVEWESNGQPENNYKTTPPVLDSDGSFFLYSKLTVDKSRWQQGNVFSCSVMHEALHNHYTQKSLSLSPGK

SEQ ID NO: 192 - protein, 98 aa, synthetic construct
  REGION 1..98: note = T.0 192
GIPPKIEALPSDISIDEGKVLTVACAFTGEPTPEVTWSCGGRKIHSQEQGRFHIENTDDLTTLIIMDVQKQDGGLYTLSLGNEFGSDSATVNIHIRSI

SEQ ID NO: 193 - protein, 98 aa, synthetic construct
  REGION 1..98: note = T.1 193
GIPPKIECLPSDISIDEGKVLTVASAFTGEPTPEVTWSTGGRKIHSQEQGRFHIENTDDLTTLIIMDVQKQDGGLYTLSLGNEFGSDSATVNIHIRSI

SEQ ID NO: 194 - protein, 98 aa, synthetic construct
  REGION 1..98: note = T.2 194
GIPPKIEALPSDISIDEGKCLTVASAFTGEPTPEVTWSTGGRKIHSQEQGRFHIENTDDLTTLIIMDVQKQDGGLYTLSLGNEFGSDSATVNIHIRSI

SEQ ID NO: 195 - protein, 98 aa, synthetic construct
  REGION 1..98: note = T.3 195
GIPPKIEALPSDISIDEGKVLTVASCFTGEPTPEVTWSTGGRKIHSQEQGRFHIENTDDLTTLIIMDVQKQDGGLYTLSLGNEFGSDSATVNIHIRSI

SEQ ID NO: 196 - protein, 98 aa, synthetic construct
  REGION 1..98: note = T.4 196
GIPPKIEALPSDISIDEGKVLCVASAFTGEPTPEVTWSTGGRKIHSQEQGRFHIENTDDLTTLIIMDVQKQDGGLYTLSLGNEFGSDSATVNIHIRSI

SEQ ID NO: 197 - protein, 103 aa, synthetic construct
  REGION 1..103: note = T.5 197
KAGIRGIPPKIECLPSDISIDEGKVLTVASAFTGEPTPEVTWSTGGRKIHSQEQGRFHIENTDDLTTLIIMDVQKQDGGLYTLSLGNEFGSDSATVNIHIRSI

SEQ ID NO: 198 - protein, 103 aa, synthetic construct
  REGION 1..103: note = T.6 198
KAGIRGIPPKIEALPSDISIDEGKVLTVACAFTGEPTPEVTWSCGGRKIHSQEQGRFHIENTDDLTTLIIMDVQKQDGGLYTLSLGNEFGSDSATVNIHIRSI

SEQ ID NO: 199 - protein, 98 aa, synthetic construct
  REGION 1..98: note = T.7 199
GIPPKIECLPSDISIDEGKVLTVASAFTGEPTPEVTWSTGGRKIHSQEQGRFHIENTDDLTTLIISDVQKQDGGLYSLSLGNEFGSDSATVNIHIRSI

SEQ ID NO: 200 - protein, 98 aa, synthetic construct
  REGION 1..98: note = T.8 200
GIPPKIECLPSDISIDEGKVLTVASAFTGEPTPEVTWSTGGRKIHSQEQGRFHIENTDDLTTLIIKDVQRQDGGLYTLTLRNEFGSDSATVNIHIRSI

SEQ ID NO: 201 - protein, 98 aa, synthetic construct
  REGION 1..98: note = T.9 201
GIWPKIECLPIDLSIDEGKVLMVASAFTGEPTPEVTWSTGGRKIHSQEQGRFHIENTDDLTTLIIMDVQKQDGGLYTLSLGMEFGSDSATVNIHIRSI

SEQ ID NO: 202 - protein, 98 aa, synthetic construct
  REGION 1..98: note = T.10 202
GIPPKIECLPIDISIDEGKVLTVASAFTGEPTPEVTWSTGGRKIHSQEQGRFHIENTDDLTTLIIKDVQKQDGGLYTLTLRNEFGSDSATVNIHIRSI

SEQ ID NO: 203 - protein, 98 aa, synthetic construct
  REGION 1..98: note = T.11 203
GIPPKIECLPSDISIDEGKVLTVASAFTGEPTPEVTWSTSGKKISSEEGGRFHIESTEDLTTLIIMDVQKQDGGVYTLSLGNDLGSDSATVNIHIRSI

SEQ ID NO: 204 - protein, 98 aa, synthetic construct
  REGION 1..98: note = T.12 204
GIPPKIECLPSDISIDEGKVLTVASAFTGEPTPEVTWSTGGRKIHSEEGGRFHIESTEDLTTLIIMDVQKQDGGVYTLSLGNEFGSDSATVNIHIRSI

SEQ ID NO: 205 - protein, 98 aa, synthetic construct
  REGION 1..98: note = T.13 205
GIPPKIECLPSDISIDEGKVLTVASAFTGEPTPEVTWSTGGRKIHSQEQGRFHIESTEDLTTLIIMDVQKQDGGVYTLSLGNEFGSDSATVNIHIRSI

SEQ ID NO: 206 - protein, 98 aa, synthetic construct
  REGION 1..98: note = T.14 206
GIPPKIECLPSDISIDEGKVLTVASAFTGEPTPEVTWSTGGRKIHSQEQGRFHIESTEDLTTLIISDVQKQDGGLYSLSLGNEFGSDSATVNIHIRSI

SEQ ID NO: 207 - protein, 103 aa, synthetic construct
  REGION 1..103: note = T.15 207
KAGIRGIPPKIECLPSDISIDEGKVLTVASAFTGEPTPEVTWSTGGRKIHSQEQGRFHIESTEDLTTLIISDVQKQDGGLYSLSLGNEFGSDSATVNIHIRSI

SEQ ID NO: 208 - protein, 98 aa, synthetic construct
  REGION 1..98: note = T.16 208
GIPPKIECLPIDISIDEGKVLTVASAFTGEPTPEVTWSTGGRKIHSQEQGRFHIENTDDSTTLTIKDVQKQDGGLYTLTLRNEFGSDSATVNIHIRSI

SEQ ID NO: 209 - protein, 98 aa, synthetic construct
  REGION 1..98: note = T.17 209
GIPPKIECLPIDISIDEGKCLTVASAFTGEPTPEVTWSTGGRKIHSQEQGRFHIENTDDSTTLTIKDVQKQDGGLYTLTLRNEFGSDSATVNIHIRSI

SEQ ID NO: 210 - protein, 98 aa, synthetic construct
  REGION 1..98: note = T.18 210
GIPPKIECLPIDISIDEGKVLTVASCFTGEPTPEVTWSTGGRKIHSQEQGRFHIENTDDSTTLTIKDVQKQDGGLYTLTLRNEFGSDSATVNIHIRSI

SEQ ID NO: 211 - protein, 97 aa, synthetic construct
  REGION 1..97: note = O.0 211
SGAPRFLTRPKAFVVSVGKDATLSCQIVGNPTPQVSWEKDQQPVAAGARFRLAQDGDLYRLTILDLALGDSGQYVCRARNAIGEAFAAVGLQVDAEA

SEQ ID NO: 212 - protein, 98 aa, synthetic construct
  REGION 1..98: note = OL.0 212
QGSPPCFLRFPRPVRVVSGAEAELKCVVLGEPPPVVVWEKGGQQLAASERLSFPADGAEHGLLLTAALPTDAGVYVCRARNAAGEAYAAAAVTVLEPP

SEQ ID NO: 213 - protein, 97 aa, synthetic construct
  REGION 1..97: note = O.1 213
SGAPRFLTRPKAFVVSVGKDATLSCQIVGNPTPQVSWEKDQQPVAAGARFRLAQDGDLYRLTILDLALGDSGQYVCRARNAIGEAFACVGLQVDAEA

SEQ ID NO: 214 - protein, 97 aa, synthetic construct
  REGION 1..97: note = O.2 214
SGCPRFLTRPKAFVVSVGKDATLSCQIVGNPTPQVSWEKDQQPVAAGARFRLAQDGDLYRLTILDLALGDSGQYVCRARNAIGEAFAAVGLQVDAEA

SEQ ID NO: 215 - protein, 97 aa, synthetic construct
  REGION 1..97: note = O.3 215
SGAPRFLTCPKAFVVSVGKDATLSCQIVGNPTPQVSWEKDQQPVAAGARFRLAQDGDLYRLTILDLALGDSGQYVCRARNAIGEAFAAVGLQVDAEA

SEQ ID NO: 216 - protein, 97 aa, synthetic construct
  REGION 1..97: note = O.4 216
SGAPRFLTRPKAFVVSVGKDATLSSQIVGNPTPQVSWEKDQQPVAAGARFRLAQDGDLYRLTILDLALGDSGQYVSRARNAIGEAFACVGLQVDAEA

SEQ ID NO: 217 - protein, 97 aa, synthetic construct
  REGION 1..97: note = O.5 217
SGCPRFLTRPKAFVVSVGKDATLSSQIVGNPTPQVSWEKDQQPVAAGARFRLAQDGDLYRLTILDLALGDSGQYVSRARNAIGEAFAAVGLQVDAEA

SEQ ID NO: 218 - protein, 97 aa, synthetic construct
  REGION 1..97: note = O.6 218
SGAPRFLTCPKAFVVSVGKDATLSSQIVGNPTPQVSWEKDQQPVAAGARFRLAQDGDLYRLTILDLALGDSGQYVSRARNAIGEAFAAVGLQVDAEA

SEQ ID NO: 219 - protein, 97 aa, synthetic construct
  REGION 1..97: note = O.7 219
SGAPRFKTRPKAFVVSVGKDATLSSQIVGNPTPQVSWEKDQQPVAAGARFRLAQDGDLYRLKILDLALGDSGQYVSRARNAIGEAFACVGLQVDAEA

SEQ ID NO: 220 - protein, 97 aa, synthetic construct
  REGION 1..97: note = O.8 220
SGAPRFKTRPKAFVVSVGKDATLSSQIVGNPTPQVSWEKDQQPVAAGARFRLAQDGDLYRLHILDLALGDSGQYVSRARNAIGEAFACVGLQVDAEA

SEQ ID NO: 221 - protein, 97 aa, synthetic construct
  REGION 1..97: note = O.9 221
SGAPRFLTRPLAFVVSVGKDATLSSQIVGNPTPQVSWEKDQQPVAAGARFRLAQDGDLYRLKILDLALGDSGQYVSRARNAIGEAFACVGLQVDAEA

SEQ ID NO: 222 - protein, 97 aa, synthetic construct
  REGION 1..97: note = O.10 222
SGAPRFLTRPLAFVVSVGKDATLSSQIVGNPTPQVSWEKDQQPVAAGARFRLAQDGDLYRLHILDLALGDSGQYVSRARNAIGEAFACVGLQVDAEA

SEQ ID NO: 223 - protein, 102 aa, synthetic construct
  REGION 1..102: note = O.11 223
DQPQFSGAPRFLTRPKAFVVSVGKDATLSSQIVGNPTPQVSWEKDQQPVAAGARFRLAQDGDLYRLTILDLALGDSGQYVSRARNAIGEAFACVGLQVDAEA

SEQ ID NO: 224 - protein, 102 aa, synthetic construct
  REGION 1..102: note = O.12 224
DQPQFSGAPRFKTRPKAFVVSVGKDATLSSQIVGNPTPQVSWEKDQQPVAAGARFRLAQDGDLYRLKILDLALGDSGQYVSRARNAIGEAFACVGLQVDAEA

SEQ ID NO: 225 - protein, 102 aa, synthetic construct
  REGION 1..102: note = O.13 225
DQPQFSGAPRFKTRPKAFVVSVGKDATLSSQIVGNPTPQVSWEKDQQPVAAGARFRLAQDGDLYRLHILDLALGDSGQYVSRARNAIGEAFACVGLQVDAEA

SEQ ID NO: 226 - protein, 102 aa, synthetic construct
  REGION 1..102: note = O.14 226
DQPQFSGAPRFRTRPKAFVVSVGKDATLSSQIVGNPTPQVSWEKDQQPVAAGARFRLAQDGDLYRLKILDLALGDSGQYVSRARNAIGEAFACVGLQVDAEA

SEQ ID NO: 227 - protein, 102 aa, synthetic construct
  REGION 1..102: note = O.15 227
DQPQFSGAPRFRTRPKAFVVSVGKDATLSSQIVGNPTPQVSWEKDQQPVAAGARFRLAQDGDLYRLHILDLALGDSGQYVSRARNAIGEAFACVGLQVDAEA

SEQ ID NO: 228 - protein, 102 aa, synthetic construct
  REGION 1..102: note = O.16 228
DQPQFSGAPRFLTRPKAFVVSVGKDATLSCQIVGNPTPQVSWEKDQQPVAAGARFRLAQDGDLYRLTILDLALGDSGQYVCRARNAIGEAFAAVGLQVDAEA

SEQ ID NO: 229 - protein, 98 aa, synthetic construct
  REGION 1..98: note = OL.1 229
QGSPPEFLRFPRPVRVVSGAEAELKCVVLGEPPPVVVWEKGGQQLAASERLSFPADGAEHGLLLTAALPTDAGCYVCRARNAAGEAYAAAAVTVLEPP

SEQ ID NO: 230 - protein, 98 aa, synthetic construct
  REGION 1..98: note = OL.2 230
QGSPPEFLRFPRPVRVVSGAEAELKCVVLGEPPPVVVWEKGGQQLAASERLSFPADGAEHGLLLTAALPTDAGVYVCRARNAACEAYAAAAVTVLEPP

SEQ ID NO: 231 - protein, 98 aa, synthetic construct
  REGION 1..98: note = OL.3 231
QGSPPEFLRFPRPVRVVSGAEAELKCVVLGEPPPVVVWEKGGQQLAASERLSFPADGAEHGLLLTAALPTDAGVYVCRARNAAGECYAAAAVTVLEPP

SEQ ID NO: 232 - protein, 98 aa, synthetic construct
  REGION 1..98: note = OL.4 232
QGSPPEFLRFPRPVRVVSGAEAELKSVVLGEPPPVVVWEKGGQQLAASERLSFPADGAEHGLLLTAALPTDAGCYVSRARNAAGEAYAAAAVTVLEPP

SEQ ID NO: 233 - protein, 98 aa, synthetic construct
  REGION 1..98: note = OL.5 233
QGSPPEFLRFPRPVRVVSGAEAELKSVVLGEPPPVVVWEKGGQQLAASERLSFPADGAEHGLLLTAALPTDAGVYVSRARNAACEAYAAAAVTVLEPP

SEQ ID NO: 234 - protein, 98 aa, synthetic construct
  REGION 1..98: note = OL.6 234
QGSPPEFLRFPRPVRVVSGAEAELKSVVLGEPPPVVVWEKGGQQLAASERLSFPADGAEHGLLLTAALPTDAGVYVSRARNAAGECYAAAAVTVLEPP

SEQ ID NO: 235 - protein, 97 aa, synthetic construct
  REGION 1..97: note = O.17 235
SGAPRFLTRPKSYTVSVGKDASLSSQIVGNPTPQVSWEKDQQPVAAGARFRLAQDGDLYRLKILDLALGDSGQYVSRARNAIGEAFACVGLQVDAEA

SEQ ID NO: 236 - protein, 97 aa, synthetic construct
  REGION 1..97: note = O.18 236
SEAPRFLTRPLAFVVSEGKDATLSSQIVGDPPPEVTWEKDQQPITAGARFRLAQDGDVYRLEILDLQLSDSGQYVSRARNAIGEAFACVGLQVDAEG

SEQ ID NO: 237 - protein, 97 aa, synthetic construct
  REGION 1..97: note = O.19 237
SGAPRFLTRPLAFVVSVGKLAMLSSQIVGNPTPQVSWEKDQQPVAAGARFRLLQDGDLYRLKILDLALGDSGQYVSRARNAIGEAFACVGLQVDAEA

SEQ ID NO: 238 - protein, 97 aa, synthetic construct
  REGION 1..97: note = O.20 238
SGAPRFLTRPLAFVVSVGKDATLSSQIVGNPTPQVSWEKDKQPVTAGARFRLAQDGDLYRLKILDLQLSDSGQYVSRARNAIGEAFACLGLQVDAEA

SEQ ID NO: 239 - protein, 97 aa, synthetic construct
  REGION 1..97: note = O.21 239
SGAPRFLTRPLAFVVSVGKDATLSSQIVGNPTPQVSWEKDQLPVTAGARFRLAQDGDLYRLKILDLTLSDSGQYVSRARNAIGEAFACVGLEVGAEA

SEQ ID NO: 240 - protein, 97 aa, synthetic construct
  REGION 1..97: note = O.22 240
SGAPRFLTRPLSYVVSVGKDASLSSQIVGNPTPQVSWEKDQLPVTAGARFRLAQDGDLYRLKILDLQLSDSGQYVSRARNAIGEAFACVGLEVGAEA

SEQ ID NO: 241 - protein, 102 aa, synthetic construct
  REGION 1..102: note = O.23 241
DQPQFSGAPRFLTRPLSYVVSVGKDASLSSQIVGNPTPQVSWEKDQLPVTAGARFRLAQDGDLYRLKILDLQLSDSGQYVSRARNAIGEAFACVGLEVGAEA

SEQ ID NO: 242 - protein, 97 aa, synthetic construct
  REGION 1..97: note = O.24 242
SGAPRFLTRPKAFVVSVGKDATLSSQIVGNPFPQVSWEKDKQPVTAGVRFRLAQDGDLYRLKILDLQLSDSGQYVSRARNAIGEAFACLGLQVDAEA

SEQ ID NO: 243 - protein, 97 aa, synthetic construct
  REGION 1..97: note = O.25 243
SGAPRFLTRPKASVVSVGKDATLSSQIVGNPFPQVSWEKDKQPVTAGVRFRLAQDGDLYRLKILDLQLSDSGQYVSRARNAHGEAFACLGLQVDAEA

SEQ ID NO: 244 - protein, 97 aa, synthetic construct
  REGION 1..97: note = O.26 244
SGCPRFLTRPKASVVSVGKDATLSSQIVGNPFPQVSWEKDKQPVTAGVRFRLAQDGDLYRLKILDLQLSDSGQYVSRARNAHGEAFACLGLQVDAEA

SEQ ID NO: 245 - protein, 97 aa, synthetic construct
  REGION 1..97: note = O.27 245
SGAPRFLTCPKASVVSVGKDATLSSQIVGNPFPQVSWEKDKQPVTAGVRFRLAQDGDLYRLKILDLQLSDSGQYVSRARNAHGEAFACLGLQVDAEA

SEQ ID NO: 246 - protein, 97 aa, synthetic construct
  REGION 1..97: note = O.28 246
SGAPRFLTRPKASVVSVGKDATLSCQIVGNPFPQVSWEKDKQPVTAGVRFRLAQDGDLYRLKILDLQLSDSGQYVCRARNAHGEAFACLGLQVDAEA

SEQ ID NO: 247 - protein, 97 aa, synthetic construct
  REGION 1..97: note = O.29 247
SGCPRFLTRPKASVVSVGKDATLSCQIVGNPFPQVSWEKDKQPVTAGVRFRLAQDGDLYRLKILDLQLSDSGQYVCRARNAHGEAFACLGLQVDAEA

SEQ ID NO: 248 - protein, 97 aa, synthetic construct
  REGION 1..97: note = O.30 248
SGAPRFLTCPKASVVSVGKDATLSCQIVGNPFPQVSWEKDKQPVTAGVRFRLAQDGDLYRLKILDLQLSDSGQYVCRARNAHGEAFACLGLQVDAEA

SEQ ID NO: 249 - protein, 97 aa, synthetic construct
  REGION 1..97: note = O.31 249
SGAPRFLTRPKASVVSVGKDATLSSQIVGNPFPQVSWEKDKQPVTAGVRFRLAQDGDLYRLKILDCQLSDSGQYVSRARNAHGEAFACLGLQCDAEA

SEQ ID NO: 250 - protein, 97 aa, synthetic construct
  REGION 1..97: note = O.32 250
SGCPRFLTRPKASVVSVGKDATLSSQIVGNPFPQVSWEKDKQPVTAGVRFRLAQDGDLYRLKILDCQLSDSGQYVSRARNAHGEAFACLGLQCDAEA

SEQ ID NO: 251 - protein, 97 aa, synthetic construct
  REGION 1..97: note = O.33 251
SGAPRFLTCPKASVVSVGKDATLSSQIVGNPFPQVSWEKDKQPVTAGVRFRLAQDGDLYRLKILDCQLSDSGQYVSRARNAHGEAFACLGLQCDAEA

SEQ ID NO: 252 - protein, 982 aa, synthetic construct
  REGION 1..982: note = AMG-757
QVQLQESGPGLVKPSETLSLTCTVSGGSISSYYWSWIRQPPGKCLEWIGYVYYSGTTNYNPSLKSRVTISVDTSKNQFSLKLSSVTAADTAVYYCASIAVTGFYFDYWGQGTLVTVSSGGGGSGGGGSGGGGSEIVLTQSPGTLSLSPGERVTLSCRASQRVNNNYLAWYQQRPGQAPRLLIYGASSRATGIPDRFSGSGSGTDFTLTISRLEPEDFAVYYCQQYDRSPLTFGCGTKLEIKSGGGGSEVQLVESGGGLVQPGGSLKLSCAASGFTFNKYAMNWVRQAPGKGLEWVARIRSKYNNYATYYADSVKDRFTISRDDSKNTAYLQMNNLKTEDTAVYYCVRHGNFGNSYISYWAYWGQGTLVTVSSGGGGSGGGGSGGGGSQTVVTQEPSLTVSPGGTVTLTCGSSTGAVTSGNYPNWVQQKPGQAPRGLIGGTKFLAPGTPARFSGSLLGGKAALTLSGVQPEDEAEYYCVLWYSNRWVFGGGTKLTVLGGGGDKTHTCPPCPAPELLGGPSVFLFPPKPKDTLMISRTPEVTCVVVDVSHEDPEVKFNWYVDGVEVHNAKTKPCEEQYGSTYRCVSVLTVLHQDWLNGKEYKCKVSNKALPAPIEKTISKAKGQPREPQVYTLPPSREEMTKNQVSLTCLVKGFYPSDIAVEWESNGQPENNYKTTPPVLDSDGSFFLYSKLTVDKSRWQQGNVFSCSVMHEALHNHYTQKSLSLSPGGGGSGGGGSGGGGSGGGGSGGGGSGGGGSDKTHTCPPCPAPELLGGPSVFLFPPKPKDTLMISRTPEVTCVVVDVSHEDPEVKFNWYVDGVEVHNAKTKPCEEQYGSTYRCVSVLTVLHQDWLNGKEYKCKVSNKALPAPIEKTISKAKGQPREPQVYTLPPSREEMTKNQVSLTCLVKGFYPSDIAVEWESNGQPENNYKTTPPVLDSDGSFFLYSKLTVDKSRWQQGNVFSCSVMHEALHNHYTQKSLSLSPGK

SEQ ID NO: 253 - protein, 705 aa, synthetic construct
  REGION 1..705: note = BI-764532 1
DIQMTQSPSAMSASVGDRVTITCRASQGISNYLVWFQQKPGKAPKRLIYAVSSLYSGVPSRFSGSGSGTEFTLTISSLQPEDFATYYCLQHDSYPYTFGQGTKLEIKRTVAAPSVFIFPPSDEQLKSGTASVVCLLNNFYPREAKVQWKVDNALQSGNSQESVTEQDSKDSTYSLSSTLTLSKADYEKHKVYACEVTHQGLSSPVTKSFNRGECGGGGSEGKSSGSGSESKSTEGKSSGSGSESKSTGGGGSQVQLVQSGAEVKKPGASVKVSCKASGYTFTSYYVHWVRQAPGQGLEWMVIINPGGGTTSYAQKFLGRVTMTRDTSTNTVYMELKSLRSEDTAVYYCARGEAVTGNYFYYGMDVWGQGTTVTVSSASTKGPSVFPLAPSSKSTSGGTAALGCLVKDYFPEPVTVSWNSGALTSGVHTFPAVLQSSGLYSLSSVVTVPSSSLGTQTYICNVNHKPSNTKVDKRVEPKSCDKTHTCPPCPAPEAAGGPSVFLFPPKPKDTLMISRTPEVTCVVVDVSHEDPEVKFNWYVDGVEVHNAKTKPREEQYNSTYRVVSVLTVLHQDWLNGKEYKCKVSNKALPAPIEKTISKAKGQPREPQVYTLPPSREEMTKNQVSLWCLVKGFYPSDIAVEWESNGQPENNYKTTPPVLDSDGSFFLYSKLTVDKSRWQQGNVFSCSVMHEALHNHYTQKSLSLSPG

SEQ ID NO: 254 - protein, 707 aa, synthetic construct
  REGION 1..707: note = BI-764532 2
EAVVTQEPSLTVSPGGTVTLTCRSSTGAVTTSNYANWVQEKPGQLPRGLIGGTNKRAPWVPARFSGSLLGGKAALTLSGAQPEDEAEYFCALWYSNLWVFGGGTKLTVLGQPKAAPSVTLFPPSSEELQANKATLVCLISDFYPGAVKVAWKADGSPVNTGVETTTPSKQSNNKYAASSYLSLTPEQWKSHRSYSCQVTHEGSTVEKTVAPAECSGGGGSEGKSSGSGSESKSTEGKSSGSGSESKSTGGGGSEVQLVESGGGLVQPGGSLKLSCAASGFTFNTYAMNWVRQAPGKGLEWVARIRSKYNNYATYYADSVKDRFTISRDDSKNTAYLQMNNLKTEDTAVYYCVRHGNFGNSYVSWFAYWGQGTLVTVSAASTKGPSVFPLAPSSKSTSGGTAALGCLVKDYFPEPVTVSWNSGALTSGVHTFPAVLQSSGLYSLSSVVTVPSSSLGTQTYICNVNHKPSNTKVDKRVEPKSCDKTHTCPPCPAPEAAGGPSVFLFPPKPKDTLMISRTPEVTCVVVDVSHEDPEVKFNWYVDGVEVHNAKTKPREEQYNSTYRVVSVLTVLHQDWLNGKEYKCKVSNKALPAPIEKTISKAKGQPREPQVYTLPPSREEMTKNQVSLSCAVKGFYPSDIAVEWESNGQPENNYKTTPPVLDSDGSFFLVSKLTVDKSRWQQGNVFSCSVMHEALHNRFTQKSLSLSPG

SEQ ID NO: 255 - protein, 5 aa, synthetic construct
  source 1..5: note = linker
ASTKG

SEQ ID NO: 256 - protein, 5 aa, synthetic construct
  source 1..5: note = linker
RTVAS

SEQ ID NO: 257 - protein, 118 aa, synthetic construct
  source 1..118: note = VH2-L
QVQLVESGGGVVQPGRSLRLSCAASGFTFSSYTMHWVRQAPGKGLEWVTFISYDGNNKYYADSVKGRFTISRDNSKNTLYLQMNSLRAEDTAIYYCARTGWLGPFDYWGQGTLVTVSS

SEQ ID NO: 258 - protein, 108 aa, synthetic construct
  source 1..108: note = VL2-L
EIVLTQSPGTLSLSPGERATLSCRASQSVGSSYLAWYQQKPGQAPRLLIYGAFSRATGIPDRFSGSGSGTDFTLTISRLEPEDFAVYYCQQYGSSPWTFGQGTKVEIK

SEQ ID NO: 259 - protein, 463 aa, synthetic construct
  source 1..463: note = hu6VL (D56E) -I2CVH-knob
DIQMTQSPSSLSASVGDRVTITCHASQGISGNMGWLQQKPGKAPKGLIYHGANLEEGVPSRFSGSGSGADYTLTISSLQPEDFADYYCVQYAQFPYTFGGGTKVEIKGGGSGGGGEVQLVESGGGLVQPGGSLKLSCAASGFTFNKYAMNWVRQAPGKGLEWVARIRSKYNNYATYYADSVKDRFTISRDDSKNTAYLQMNNLKTEDTAVYYCVRHGNFGNSYISYWAYWGQGTLVTVSSGCPPCPAPEAAGAPSVFLFPPKPKDTLMISRTPEVTCVVVDVSHEDPEVKFNWYVDGVEVHNAKTKPREEQYNSTYRVVSVLTVLHQDWLNGKEYKCKVSNKALPAPIEKTISKAKGQPREPQVCTLPPSREEMTKNQVSLWCLVKGFYPSDIAVEWESNGQPENNYKTTPPVLDSDGSFFLYSKLTVDKSRWQQGNVFSCSVMHEALHNHYTQKSLSLSPGK

SEQ ID NO: 260 - protein, 463 aa, synthetic construct
  source 1..463: note = hu6VL (D56S) -I2CVH-knob
DIQMTQSPSSLSASVGDRVTITCHASQGISGNMGWLQQKPGKAPKGLIYHGANLESGVPSRFSGSGSGADYTLTISSLQPEDFADYYCVQYAQFPYTFGGGTKVEIKGGGSGGGGEVQLVESGGGLVQPGGSLKLSCAASGFTFNKYAMNWVRQAPGKGLEWVARIRSKYNNYATYYADSVKDRFTISRDDSKNTAYLQMNNLKTEDTAVYYCVRHGNFGNSYISYWAYWGQGTLVTVSSGCPPCPAPEAAGAPSVFLFPPKPKDTLMISRTPEVTCVVVDVSHEDPEVKFNWYVDGVEVHNAKTKPREEQYNSTYRVVSVLTVLHQDWLNGKEYKCKVSNKALPAPIEKTISKAKGQPREPQVCTLPPSREEMTKNQVSLWCLVKGFYPSDIAVEWESNGQPENNYKTTPPVLDSDGSFFLYSKLTVDKSRWQQGNVFSCSVMHEALHNHYTQKSLSLSPGK